European Patent Application EP 4 471 137 A2, published December 4, 2024. Title: CARBOXYESTERASE BIOCATALYSTS. Applicant: GlaxoSmithKline Intellectual Property Development Limited. The sequence listing filed with the application follows.

SEQUENCE LISTING (126 sequences)

SEQ ID NO: 1 - DNA, 930 bp, Alicyclobacillus acidocaldarius
  source 1..930: mol_type = other DNA
atgccattagatcctgtgattcaacaagtcctcgatcaactgaaccgtatgccagcccctgactacaagcacttaagcgctcaacagtttcgttcacagcaatcactgtttccaccagttaagaaagaaccggtcgcagaagttcgcgaattcgacatggatctgccgggccgtaccctgaaagtccgtatgtaccgtccggaaggtgttgaaccaccatatccagcactggtttactaccatggtggcggttgggttgttggtgacctggaaacgcatgatccggtgtgtcgtgtgttggcgaaagatggacgcgcagtggtgtttagcgttgactaccgtctggcaccagaacacaagtttccagcggcagttgaagacgcgtatgatgcactgcaatggattgcagaacgtgcagccgatttccatcttgatccagcacgcattgcagttggcggcgattcagcaggcggcaacctggcggccgtgactagtattctggcgaaagaacgtggtggtccagcaattgcgtttcaactgctgatctatccctccactggttatgatccagcacatccaccagcaagtatcgaagagaatgcggagggttacctgttaaccggaggcatgatgctgtggtttcgtgaccagtacctgaacagccttgaggaactgactcacccatggtttagtccagtgctgtacccggatcttagcggtttaccaccggcgtacattgcaaccgcacagtacgatcccctgcgcgatgtcggcaaactttacgctgaagccctgaacaaagcgggcgttaaggtggagatcgagaacttcgaggatctgattcatggcttcgcgcagttctattctctgagcccaggcgcaaccaaagcactggtacgtattgccgagaaactgcgcgatgcgttggcg

SEQ ID NO: 2 - protein, 310 aa, Alicyclobacillus acidocaldarius
MPLDPVIQQVLDQLNRMPAPDYKHLSAQQFRSQQSLFPPVKKEPVAEVREFDMDLPGRTLKVRMYRPEGVEPPYPALVYYHGGGWVVGDLETHDPVCRVLAKDGRAVVFSVDYRLAPEHKFPAAVEDAYDALQWIAERAADFHLDPARIAVGGDSAGGNLAAVTSILAKERGGPAIAFQLLIYPSTGYDPAHPPASIEENAEGYLLTGGMMLWFRDQYLNSLEELTHPWFSPVLYPDLSGLPPAYIATAQYDPLRDVGKLYAEALNKAGVKVEIENFEDLIHGFAQFYSLSPGATKALVRIAEKLRDALA

SEQ ID NO: 3 - DNA, 930 bp, synthetic construct
  misc_feature 1..930: note = Description of Artificial Sequence: Syntheticpolynucleotide sequence encoding a codon optimizedcarboxyesterase enzyme
  source 1..930: mol_type = other DNA
atgccattagatcctgtgattcaacaagtcctcgatcaactgaaccgtatgccagcccctgactacaagcacttaagcgctcaacagtttcgttcacagcaatcactgtttccaccagttaagaaagaaccggtcgcagaagttcgcgaattcgacatggatctgccgggccgtaccctgaaagtccgtatgtaccgtccggaaggtgttgaaccaccatatccagcactggtttactaccatggtggcggttgggttgttggtgacctggaaacgcatgatccggtgtgtcgtgtgttggcgaaagatggacgcgcagtggtgtttagcgttgactaccgtctggcaccagaacacaagtttccagcggcagttgaagacgcgtatgatgcactgcaatggattgcagaacgtgcagccgatttccatcttgatccagcacgcattgcagttggcggcgattcagcaggcggcaacctggcggccgtgactagtattctggcgaaagaacgtggtggtccagcaattgcgtttcaactgctgatctatccctccactggttatgatccagcacatccaccagcaagtatccttgagaatgcggagggttacctgttaaccggaggcatgatgctgtggtttcgtgaccagtacctgaacagccttgaggaactgactcacccatggtttagtccagtgctgtacccggatcttagcggtttaccaccggcgtacattgcaaccgcacagtacgatcccctgcgcgatgtcggcaaactttacgctgaagccctgaacaaagcgggcgttaaggtggagatcgagaacttcgaggatctgattcatggcttcgcgcagttctattctctgagcccaggcgcaaccaaagcactggtacgtattgccgagaaactgcgcgatgcgttggcg

SEQ ID NO: 4 - protein, 310 aa, synthetic construct
  REGION 1..310: note = Description of Artificial Sequence: Syntheticpolypeptide sequence of a codon optimizedcarboxyesterase enzyme
MPLDPVIQQVLDQLNRMPAPDYKHLSAQQFRSQQSLFPPVKKEPVAEVREFDMDLPGRTLKVRMYRPEGVEPPYPALVYYHGGGWVVGDLETHDPVCRVLAKDGRAVVFSVDYRLAPEHKFPAAVEDAYDALQWIAERAADFHLDPARIAVGGDSAGGNLAAVTSILAKERGGPAIAFQLLIYPSTGYDPAHPPASILENAEGYLLTGGMMLWFRDQYLNSLEELTHPWFSPVLYPDLSGLPPAYIATAQYDPLRDVGKLYAEALNKAGVKVEIENFEDLIHGFAQFYSLSPGATKALVRIAEKLRDALA

SEQ ID NO: 5 - DNA, 930 bp, synthetic construct
  misc_feature 1..930: note = Description of Artificial Sequence: Syntheticpolynucleotide sequence encoding a codon optimizedcarboxyesterase enzyme
  source 1..930: mol_type = other DNA
atgccattagatcctgtgattcaacaagtcctcgatcaactgaaccgtatgccagcccctgactacaagcacttaagcgctcaacagtttcgttcacagcaatcactgtttccaccagttaagaaagaaccggtcgcagaagttcgcgaattcgacatggatctgccgggccgtaccctgaaagtccgtatgtaccgtccggaaggtgttgaaccaccatatccagcactggtttactaccatggtggcggttgggttgttggtgacctggaaacgcatgatccggtgtgtcgtgtgttggcgaaagatggacgcgcagtggtgtttagcgttgactaccgtctggcaccagaacacaagtttccagcggcagttgaagacgcgtatgatgcactgcaatggattgcagaacgtgcagccgatttccatcttgatccagcacgcattgcagttggcggcgattcagcaggcggcaacctggcggccgtgactagtattctggcgaaagaacgtggtggtccagcaattgcgtttcaactgctgatctatccctccactggttatgatccagcacatccaccagcaagtatcattgagaatgcggagggttacctgttaaccggaggcatgatgctgtggtttcgtgaccagtacctgaacagccttgaggaactgactcacccatggtttagtccagtgctgtacccggatcttagcggtttaccaccggcgtacattgcaaccgcacagtacgatcccctgcgcgatgtcggcaaactttacgctgaagccctgaacaaagcgggcgttaaggtggagatcgagaacttcgaggatctgattcatggcttcgcgcagttctattctctgagcccaggcgcaaccaaagcactggtacgtattgccgagaaactgcgcgatgcgttggcg

SEQ ID NO: 6 - protein, 310 aa, synthetic construct
  REGION 1..310: note = Description of Artificial Sequence: Syntheticpolypeptide sequence of a codon optimizedcarboxyesterase enzyme
MPLDPVIQQVLDQLNRMPAPDYKHLSAQQFRSQQSLFPPVKKEPVAEVREFDMDLPGRTLKVRMYRPEGVEPPYPALVYYHGGGWVVGDLETHDPVCRVLAKDGRAVVFSVDYRLAPEHKFPAAVEDAYDALQWIAERAADFHLDPARIAVGGDSAGGNLAAVTSILAKERGGPAIAFQLLIYPSTGYDPAHPPASIIENAEGYLLTGGMMLWFRDQYLNSLEELTHPWFSPVLYPDLSGLPPAYIATAQYDPLRDVGKLYAEALNKAGVKVEIENFEDLIHGFAQFYSLSPGATKALVRIAEKLRDALA

SEQ ID NO: 7 - DNA, 930 bp, synthetic construct
  misc_feature 1..930: note = Description of Artificial Sequence: Syntheticpolynucleotide sequence encoding a codon optimizedcarboxyesterase enzyme
  source 1..930: mol_type = other DNA
atgccattagatcctgtgattcaacaagtcctcgatcaactgaaccgtatgccagcccctgactacaagcacttaagcgctcaacagtttcgttcacagcaatcactgtttccaccagttaagaaagaaccggtcgcagaagttcgcgaattcgacatggatctgccgggccgtaccctgaaagtccgtatgtaccgtccggaaggtgttgaaccaccatatccagcactggtttactaccatggtggcggttgggttgttggtgacctggaaacgcatgatccggtgtgtcgtgtgttggcgaaagatggacgcgcagtggtgtttagcgttgactaccgtctggcaccagaacacaagtttccagcggcagttgaagacgcgtatgatgcactgcaatggattgcagaacgtgcagccgatttccatcttgatccagcacgcattgcagttggcggcgattcagcaggcggcaacctggcggccgtgactagtattctggcgaaagaacgtggtggtccagcaattgcgtttcaactgctgatctatccctccactggttatgatccagcacatccaccagcaagtatctatgagaatgcggagggttacctgttaaccggaggcatgatgctgtggtttcgtgaccagtacctgaacagccttgaggaactgactcacccatggtttagtccagtgctgtacccggatcttagcggtttaccaccggcgtacattgcaaccgcacagtacgatcccctgcgcgatgtcggcaaactttacgctgaagccctgaacaaagcgggcgttaaggtggagatcgagaacttcgaggatctgattcatggcttcgcgcagttctattctctgagcccaggcgcaaccaaagcactggtacgtattgccgagaaactgcgcgatgcgttggcg

SEQ ID NO: 8 - protein, 310 aa, synthetic construct
  REGION 1..310: note = Description of Artificial Sequence: Syntheticpolypeptide sequence of a codon optimizedcarboxyesterase enzyme
MPLDPVIQQVLDQLNRMPAPDYKHLSAQQFRSQQSLFPPVKKEPVAEVREFDMDLPGRTLKVRMYRPEGVEPPYPALVYYHGGGWVVGDLETHDPVCRVLAKDGRAVVFSVDYRLAPEHKFPAAVEDAYDALQWIAERAADFHLDPARIAVGGDSAGGNLAAVTSILAKERGGPAIAFQLLIYPSTGYDPAHPPASIYENAEGYLLTGGMMLWFRDQYLNSLEELTHPWFSPVLYPDLSGLPPAYIATAQYDPLRDVGKLYAEALNKAGVKVEIENFEDLIHGFAQFYSLSPGATKALVRIAEKLRDALA

SEQ ID NO: 9 - DNA, 930 bp, synthetic construct
  misc_feature 1..930: note = Description of Artificial Sequence: Syntheticpolynucleotide sequence encoding a codon optimizedcarboxyesterase enzyme
  source 1..930: mol_type = other DNA
atgccattagatcctgtgattcaacaagtcctcgatcaactgaaccgtatgccagcccctgactacaagcacttaagcgctcaacagtttcgttcacagcaatcactgtttccaccagttaagaaagaaccggtcgcagaagttcgcgaattcgacatggatctgccgggccgtaccctgaaagtccgtatgtaccgtccggaaggtgttgaaccaccatatccagcactggtttactaccatggtggcggttgggttgttggtgacctggaaacgcatgatccggtgtgtcgtgtgttggcgaaagatggacgcgcagtggtgtttagcgttgactaccgtctggcaccagaacacaagtttccagcggcagttgaagacgcgtatgatgcactgcaatggattgcagaacgtgcagccgatttccatcttgatccagcacgcattgcagttggcggcgattcagcaggcggcaacctggcggccgtgactagtattctggcgaaagaacgtggtggtccagcaattgcgtttcaactgctgatctatccctccactggttatgatccagcacatccaccagcaagtatctttgagaatgcggagggttacctgttaaccggaggcatgatgctgtggtttcgtgaccagtacctgaacagccttgaggaactgactcacccatggtttagtccagtgctgtacccggatcttagcggtttaccaccggcgtacattgcaaccgcacagtacgatcccctgcgcgatgtcggcaaactttacgctgaagccctgaacaaagcgggcgttaaggtggagatcgagaacttcgaggatctgattcatggcttcgcgcagttctattctctgagcccaggcgcaaccaaagcactggtacgtattgccgagaaactgcgcgatgcgttggcg

SEQ ID NO: 10 - protein, 310 aa, synthetic construct
  REGION 1..310: note = Description of Artificial Sequence: Syntheticpolypeptide sequence of a codon optimizedcarboxyesterase enzyme
MPLDPVIQQVLDQLNRMPAPDYKHLSAQQFRSQQSLFPPVKKEPVAEVREFDMDLPGRTLKVRMYRPEGVEPPYPALVYYHGGGWVVGDLETHDPVCRVLAKDGRAVVFSVDYRLAPEHKFPAAVEDAYDALQWIAERAADFHLDPARIAVGGDSAGGNLAAVTSILAKERGGPAIAFQLLIYPSTGYDPAHPPASIFENAEGYLLTGGMMLWFRDQYLNSLEELTHPWFSPVLYPDLSGLPPAYIATAQYDPLRDVGKLYAEALNKAGVKVEIENFEDLIHGFAQFYSLSPGATKALVRIAEKLRDALA

SEQ ID NO: 11 - DNA, 930 bp, synthetic construct
  misc_feature 1..930: note = Description of Artificial Sequence: Syntheticpolynucleotide sequence encoding a codon optimizedcarboxyesterase enzyme
  source 1..930: mol_type = other DNA
atgccattagatcctgtgattcaacaagtcctcgatcaactgaaccgtatgccagcccctgactacaagcacttaagcgctcaacagtttcgttcacagcaatcactgtttccaccagttaagaaagaaccggtcgcagaagttcgcgaattcgacatggatctgccgggccgtaccctgaaagtccgtatgtaccgtccggaaggtgttgaaccaccatatccagcactggtttactaccatggtggcggttgggttgttggtgacctggaaacgcatgatccggtgtgtcgtgtgttggcgaaagatggacgcgcagtggtgtttagcgttgactaccgtctggcaccagaacacaagtttccagcggcagttgaagacgcgtatgatgcactgcaatggattgcagaacgtgcagccgatttccatcttgatccagcacgcattgcagttggcggcgattcagcaggcggcaacctggcggccgtgactagtattctggcgaaagaacgtggtggtccggcaattgcgtttcaactgctgatctatccctccactggttatgatccagcacatccaccagcaagtatcatggagaatgcggagggttacctgttaaccggaggcatgatgctgtggtttcgtgaccagtacctgaacagccttgaggaactgactcacccatggtttagtccagtgctgtacccggatcttagcggtttaccaccggcgtacattgcaaccgcacagtacgatcccctgcgcgatgtcggcaaactttacgctgaagccctgaacaaagcgggcgttaaggtggagatcgagaacttcgaggatctgattcatggcttcgcgcagttctattctctgagcccaggcgcaaccaaagcactggtacgtattgccgagaaactgcgcgatgcgttggcg

SEQ ID NO: 12 - protein, 310 aa, synthetic construct
  REGION 1..310: note = Description of Artificial Sequence: Syntheticpolypeptide sequence of a codon optimizedcarboxyesterase enzyme
MPLDPVIQQVLDQLNRMPAPDYKHLSAQQFRSQQSLFPPVKKEPVAEVREFDMDLPGRTLKVRMYRPEGVEPPYPALVYYHGGGWVVGDLETHDPVCRVLAKDGRAVVFSVDYRLAPEHKFPAAVEDAYDALQWIAERAADFHLDPARIAVGGDSAGGNLAAVTSILAKERGGPAIAFQLLIYPSTGYDPAHPPASIMENAEGYLLTGGMMLWFRDQYLNSLEELTHPWFSPVLYPDLSGLPPAYIATAQYDPLRDVGKLYAEALNKAGVKVEIENFEDLIHGFAQFYSLSPGATKALVRIAEKLRDALA

SEQ ID NO: 13 - DNA, 930 bp, synthetic construct
  misc_feature 1..930: note = Description of Artificial Sequence: Syntheticpolynucleotide sequence encoding a codon optimizedcarboxyesterase enzyme
  source 1..930: mol_type = other DNA
atgccattagatcctgtgattcaacaagtcctcgatcaactgaaccgtatgccagcccctgactacaagcacttaagcgctcagcagtttcgttcacagcaatcactgttgccaccagttaagaaagaaccggtcgcagaagttcgcgaattcgacatggatctgccgggccgtaccctgaaagtccgtatgtaccgtccggaaggtgttgaaccaccatatccagcactggtttactaccatggtggcggttgggttgttggtgacctggaaacgcatgatccggtgtgtcgtgtgttggcgaaagatggacgcgcagtggtgtttagcgttgactaccgtctggcaccagaacacaagtttccagcggcagttgaagacgcgtatgatgcactgcaatggattgcagaacgtgcagccgatttccatcttgatccagcacgcattgcagttggcggcgattcagcaggcggcaacctggcggccgtgactagtattctggcgaaagaacgtggtggtccagcaattgcgtttcaactgctgatctatccctttactggttatgatccagcacatccaccagcaagtatccttgagaatgcggagggttacctgttagagcatggcatgatgctgtggtttcgtgaccagtacctgaacagccttgaggaactgactcacccatggtttagtccagtgctgtacccggatcttagcggtttaccaccggcgtacattgcaaccgcacagtacgatcccctgcgcgatgtcggcaaactttacgctgaagccctgaacaaagcgggcgttaaggtggagatcgagaacttcgaggatctgattcatggcttcgcgcaattttattctctgagcccaggcgcaaccaaagcactggtacgtattgccgagaaactgcgcgatgcgttggcg

SEQ ID NO: 14 - protein, 310 aa, synthetic construct
  REGION 1..310: note = Description of Artificial Sequence: Syntheticpolypeptide sequence of a codon optimizedcarboxyesterase enzyme
MPLDPVIQQVLDQLNRMPAPDYKHLSAQQFRSQQSLLPPVKKEPVAEVREFDMDLPGRTLKVRMYRPEGVEPPYPALVYYHGGGWVVGDLETHDPVCRVLAKDGRAVVFSVDYRLAPEHKFPAAVEDAYDALQWIAERAADFHLDPARIAVGGDSAGGNLAAVTSILAKERGGPAIAFQLLIYPFTGYDPAHPPASILENAEGYLLEHGMMLWFRDQYLNSLEELTHPWFSPVLYPDLSGLPPAYIATAQYDPLRDVGKLYAEALNKAGVKVEIENFEDLIHGFAQFYSLSPGATKALVRIAEKLRDALA

SEQ ID NO: 15 - DNA, 930 bp, synthetic construct
  misc_feature 1..930: note = Description of Artificial Sequence: Syntheticpolynucleotide sequence encoding a codon optimizedcarboxyesterase enzyme
  source 1..930: mol_type = other DNA
atgccattagatcctgtgattcaacaagtcctcgatcaactgaaccgtatgccagcccctgactacaagcacttaagcgctcagcagtttcgttcacagcaatcactgtttccaccagttaagaaagaaccggtcgcagaagttcgcgaattcgacatggatctgccgggccgtaccctgaaagtccgtatgtaccgtccggaaggtgttgaaccaccatatccagcactggtttactaccatggtggcggttgggttgttggtgacctggaaacgcatgatccggtgtgtcgtgtgttggcgaaagatggacgcgcagtggtgtttagcgttgactaccgtctggcaccagaacacaagtttccagcggcagttgaagacgcgtatgatgcactgcaatggattgcagaacgtgcagccgatttccatcttgatccagcacgcattgcagttggcggcgattcagcaggcggcaacctggcggccgtgactagtattctggcgaaagaacgtggtggtccagcaattgcgtttcaactgctgatctatccctttactggttatgatccagcacatccaccagcaagtatccttgagaatgcggagggttacctgttaaccggaggcatgatgctgtggtttcgtgaccagtacctgaacagccttgaggaactgactcacccatggtttagtccagtgctgtacccggatcttagcggtttaccaccggcgtacattgcaaccgcacagtacgatcccctgcgcgatgtcggcaaactttacgctgaagccctgaacaaagcgggcgttaaggtggagatcgagaacttcgaggatctgattcatggcttcgcgcagttctattctctgagcccaggcgcaaccaaggcactggtacgtattgccgagaaactgcgcgatgcgttggcg

SEQ ID NO: 16 - protein, 310 aa, synthetic construct
  REGION 1..310: note = Description of Artificial Sequence: Syntheticpolypeptide sequence of a codon optimizedcarboxyesterase enzyme
MPLDPVIQQVLDQLNRMPAPDYKHLSAQQFRSQQSLFPPVKKEPVAEVREFDMDLPGRTLKVRMYRPEGVEPPYPALVYYHGGGWVVGDLETHDPVCRVLAKDGRAVVFSVDYRLAPEHKFPAAVEDAYDALQWIAERAADFHLDPARIAVGGDSAGGNLAAVTSILAKERGGPAIAFQLLIYPFTGYDPAHPPASILENAEGYLLTGGMMLWFRDQYLNSLEELTHPWFSPVLYPDLSGLPPAYIATAQYDPLRDVGKLYAEALNKAGVKVEIENFEDLIHGFAQFYSLSPGATKALVRIAEKLRDALA

SEQ ID NO: 17 - DNA, 930 bp, synthetic construct
  misc_feature 1..930: note = Description of Artificial Sequence: Syntheticpolynucleotide sequence encoding a codon optimizedcarboxyesterase enzyme
  source 1..930: mol_type = other DNA
atgccattagatcctgtgattcaacaagtcctcgatcaactgaaccgtatgccagcccctgactacaagcacttaagcgctcaacagtttcgttcacagcaatcactgttgccaccagttaagaaagaaccggtcgcagaagttcgcgaattcgacatggatctgccgggccgtaccctgaaagtccgtatgtaccgtccggaaggtgttgaaccaccatatcgggcactggtttactaccatggtggcggttgggttgttggtgacctggaaacgcatgatccggtgtgtcgtgtgttggcgaaagatggacgcgcagtggtgtttagcgttgactaccgtctggcaccagaacacaagtttccagcggcagttgaagacgcgtatgatgcactgcaatggattgcagaacgtgcagccgatttccatcttgatccagcacgcattgcagttggcggcgattcagcaggcggcaacctggcggccgtgactagtattctggcgaaagaacgtggtggtccagcaattgcgtttcaactgctgatctatccctttactggttatgatccagcacatccaccagcaagtatccttgagaatgcggagggttacctgttaacgcatggcatgatgctgtggtttcgtgaccagtacctgaacagccttgaggaactgactcacccatggtttagtccagtgctgtacccggatcttagcggtttaccaccggcgtacattgcaaccgcacagtacgatcccctgcgcgatgtcggcaaactttacgctgaagccctgaacaaagcgggcgttaaggtggagatcgagaacttcgaggatctgattcatggcttcgcgcagttctattctctgagcccaggcgcaaccctcgcactggtacgtattgccgagaaactgcgcgatgcgttggcg

SEQ ID NO: 18 - protein, 310 aa, synthetic construct
  REGION 1..310: note = Description of Artificial Sequence: Syntheticpolypeptide sequence of a codon optimizedcarboxyesterase enzyme
MPLDPVIQQVLDQLNRMPAPDYKHLSAQQFRSQQSLLPPVKKEPVAEVREFDMDLPGRTLKVRMYRPEGVEPPYRALVYYHGGGWVVGDLETHDPVCRVLAKDGRAVVFSVDYRLAPEHKFPAAVEDAYDALQWIAERAADFHLDPARIAVGGDSAGGNLAAVTSILAKERGGPAIAFQLLIYPFTGYDPAHPPASILENAEGYLLTHGMMLWFRDQYLNSLEELTHPWFSPVLYPDLSGLPPAYIATAQYDPLRDVGKLYAEALNKAGVKVEIENFEDLIHGFAQFYSLSPGATLALVRIAEKLRDALA

SEQ ID NO: 19 - DNA, 930 bp, synthetic construct
  misc_feature 1..930: note = Description of Artificial Sequence: Syntheticpolynucleotide sequence encoding a codon optimizedcarboxyesterase enzyme
  source 1..930: mol_type = other DNA
atgccattagatcctgtgattcaacaagtcctcgatcaactgaaccgtatgccagcccctgactacaagcacttaagcgctcaacagtttcgttcacagcaatcactgttcccaccagttaagaaagaaccggtcgcagaagttcgcgaattcgacatggatctgccgggccgtaccctgaaagtccgtatgtaccgaccggaaggtgttgaaccaccatatccggcactggtttactaccatggtggcggttgggttgttggtgacctggaaacgcatgatccggtgtgtcgtgtgttggcgaaagatggacgcgcagtggtgtttagcgttgactaccgtctggcaccagaacacaagtttccagcggcagttgaagacgcgtatgatgcactgcaatggattgcagaacgtgcagccgatttccatcttgatccagcacgcattgcagttggcggcgattcagcaggcggcaacctggcggccgtgactagtattctggcgaaagaacgtggtggtccagcaattgcgtttcaactgctgatctatccctttactggttatgatccagcacatccaccagcaagtatccttgagaatgcggagggttacctgttagagcatggcatgatgctgtggtttcgtgaccagtacctgaacagccttgaggaactgactcacccatggtttagtccagtgctgtacccggatcttagcggtttaccaccggcgtacattgcaaccgcacagtacgatcccctgcgcgatgtcggcaaactttacgctgaagccctgaacaaagcgggcgttaaggtggagatcgagaacttcgaggatctgattcatggcttcgcgcagttctattctctgagcccaggcgcaaccaaggcactggtacgtattgccgagaaactgcgcgatgcgttggcg

SEQ ID NO: 20 - protein, 310 aa, synthetic construct
  REGION 1..310: note = Description of Artificial Sequence: Syntheticpolypeptide sequence of a codon optimizedcarboxyesterase enzyme
MPLDPVIQQVLDQLNRMPAPDYKHLSAQQFRSQQSLFPPVKKEPVAEVREFDMDLPGRTLKVRMYRPEGVEPPYPALVYYHGGGWVVGDLETHDPVCRVLAKDGRAVVFSVDYRLAPEHKFPAAVEDAYDALQWIAERAADFHLDPARIAVGGDSAGGNLAAVTSILAKERGGPAIAFQLLIYPFTGYDPAHPPASILENAEGYLLEHGMMLWFRDQYLNSLEELTHPWFSPVLYPDLSGLPPAYIATAQYDPLRDVGKLYAEALNKAGVKVEIENFEDLIHGFAQFYSLSPGATKALVRIAEKLRDALA

SEQ ID NO: 21 - DNA, 930 bp, synthetic construct
  misc_feature 1..930: note = Description of Artificial Sequence: Syntheticpolynucleotide sequence encoding a codon optimizedcarboxyesterase enzyme
  source 1..930: mol_type = other DNA
atgccattagatcctgtgattcaacaagtcctcgatcaactgaaccgtatgccagcccctgactacaagcacttaagcgctcaacagtttcgttcacagcaacacctgtttccaccagttaagaaagaaccggtcgcagaagttcgcgaattcgacatggatctgccgggccgtaccctgaaagtccgtatgtaccgcccggaaggtgttgaaccaccatatccagcactggtttactaccatggtggcggttgggttgttggtgacctggaaacgcatgatccggtgtgtcgtgtgttggcgaaagatggacgcgcagtggtgtttagcgttgactaccgtctggcaccagaacacaagtttccagcggcagttgaagacgcgtatgatgcactgcaatggattgcagaacgtgcagccgatttccatcttgatccagcacgcattgcagttggcggcgattcagcaggcggcaacctggcggccgtgactagtattctggcgaaagaacgtggtggtccagcaattgcgtttcaactgctgatctatccctttactggttatgatccagcacatccaccagcaagtatccttgagaatgcggagggttacctgttaaccggaggcatgatgctgtggtttcgtgaccagtacctgaacagccttgaggaactgactcacccatggtttagtccagtgctgtacccggatcttagcggtttaccaccggcgtacattgcaaccgcacagtacgatcccctgcgcgatgtcggcaaactttacgctgaagccctgaacaaagcgggcgttaaggtggagatcgagaacttcgaggatctgattcatggcttcgcgcagttctattctctgagcccaggcgcaaccaaagcactggtacgtattgccgagaaactgcgcgatgcgttggcg

SEQ ID NO: 22 - protein, 310 aa, synthetic construct
  REGION 1..310: note = Description of Artificial Sequence: Syntheticpolypeptide sequence of a codon optimizedcarboxyesterase enzyme
MPLDPVIQQVLDQLNRMPAPDYKHLSAQQFRSQQHLFPPVKKEPVAEVREFDMDLPGRTLKVRMYRPEGVEPPYPALVYYHGGGWVVGDLETHDPVCRVLAKDGRAVVFSVDYRLAPEHKFPAAVEDAYDALQWIAERAADFHLDPARIAVGGDSAGGNLAAVTSILAKERGGPAIAFQLLIYPFTGYDPAHPPASILENAEGYLLTGGMMLWFRDQYLNSLEELTHPWFSPVLYPDLSGLPPAYIATAQYDPLRDVGKLYAEALNKAGVKVEIENFEDLIHGFAQFYSLSPGATKALVRIAEKLRDALA

SEQ ID NO: 23 - DNA, 930 bp, synthetic construct
  misc_feature 1..930: note = Description of Artificial Sequence: Syntheticpolynucleotide sequence encoding a codon optimizedcarboxyesterase enzyme
  source 1..930: mol_type = other DNA
atgccattagatcctgtgattcaacaagtcctcgatcaactgaaccgtatgccagcacctgactacaagcacttaagcgctcaacagtttcgttcacagcaatcactgtttccaccagttaagaaagaaccggtcgcagaagttcgcgaattcgacatggatctgccgggccgtaccctgaaagtccgtatgtaccgtccggaaggtgttgaaccaccatatccagcactggtttactaccatggtggcggttgggttgttggtgacctggaaacgcatgatccggtgtgtcgtgtgttggcgaaagatggacgcgcagtggtgtttagcgttgactaccgtctggcaccagaacacaagtttccagcggcagttgaagacgcgtatgatgcactgcaatggattgcagaacgtgcagccgatttccatcttgatccagcacgcattgcagttggcggcgattcagcaggcggcaacctggcggccgtgactagtattctggcgaaagaacgtggtggtccagcaattgcgtttcaactgctgatctatcccatgactggttatgatccagcacatccaccagcaagtatccttgagaatgcggagggttacctgttagagggaggcatgatgctgtggtttcgtgaccagtacctgaacagccttgaggaactgactcacccatggtttagtccagtgctgtacccggatcttagcggtttaccaccggcgtacattgcaaccgcacagtacgatcccctgcgcgatgtcggcaaactttacgctgaagccctgaacaaagcgggcgttaaggtggagatcgagaacttcgaggatctgattcatggcttcgcgcagttctattctctgagcccaggcgcaaccgtcgcactggtacgtattgccgagaaactgcgcgatgcgttggcg

SEQ ID NO: 24 - protein, 310 aa, synthetic construct
  REGION 1..310: note = Description of Artificial Sequence: Syntheticpolypeptide sequence of a codon optimizedcarboxyesterase enzyme
MPLDPVIQQVLDQLNRMPAPDYKHLSAQQFRSQQSLFPPVKKEPVAEVREFDMDLPGRTLKVRMYRPEGVEPPYPALVYYHGGGWVVGDLETHDPVCRVLAKDGRAVVFSVDYRLAPEHKFPAAVEDAYDALQWIAERAADFHLDPARIAVGGDSAGGNLAAVTSILAKERGGPAIAFQLLIYPMTGYDPAHPPASILENAEGYLLEGGMMLWFRDQYLNSLEELTHPWFSPVLYPDLSGLPPAYIATAQYDPLRDVGKLYAEALNKAGVKVEIENFEDLIHGFAQFYSLSPGATVALVRIAEKLRDALA

SEQ ID NO: 25 - DNA, 930 bp, synthetic construct
  misc_feature 1..930: note = Description of Artificial Sequence: Syntheticpolynucleotide sequence encoding a codon optimizedcarboxyesterase enzyme
  source 1..930: mol_type = other DNA
atgccattagatcctgtgattcaacaagtcctcgatcaactgaaccgtatgccagcccctgactacaagcacttaagcccgcaacagttgcgttcacagcaatcactgtttccaccagttaagaaagaaccggtcgcagaagttcgcgaattcgacatggatctgccgggtcgtaccctgaaagtccgtatgtaccgtccggaaggtgttgaaccaccatatccagcactggtttactaccatggtggcggttgggttgttggtgacctggaaacgcatgatccggtgtgtcgtgtgttggcgaaatggggacgcgcagtggtgtttagcgttgactaccgtctggcaccagaacacaagtttccagcggcagttgaagacgcgtatgatgcactgcaatggattgcagaacgtgcagccgatttccatcttgatccagcacgcattgcagttggcggcgattcagcaggcggcaacctggcggccgtgactagtattctggcgaaagaacgtggtggtccagcaattgcgtttcaactgctgatctatccctccactggttatgatccagcacatccaccagcaagtatcattgagaatgcggagggttacctgttaaccggaggcatgatgctgtggtttcgtgaccagtacctgaacagccttgaggaactgactcacccatggtttagtccagtgctgtacccggatcttagcggtttaccaccggcgtacattgcaaccgcacagtacgatcccctgcgcgatgtcggcaaactttacgctgaagccctgaacaaagcgggcgttaaggtggagatcgagaacttcgaggatctgattcatggcttcgcggggttctattctctgagcccaggcgcaaccaaagcactggtacgtattgccgagaaactgcgcgatgcgttggcg

SEQ ID NO: 26 - protein, 310 aa, synthetic construct
  REGION 1..310: note = Description of Artificial Sequence: Syntheticpolypeptide sequence of a codon optimizedcarboxyesterase enzyme
MPLDPVIQQVLDQLNRMPAPDYKHLSPQQLRSQQSLFPPVKKEPVAEVREFDMDLPGRTLKVRMYRPEGVEPPYPALVYYHGGGWVVGDLETHDPVCRVLAKWGRAVVFSVDYRLAPEHKFPAAVEDAYDALQWIAERAADFHLDPARIAVGGDSAGGNLAAVTSILAKERGGPAIAFQLLIYPSTGYDPAHPPASIIENAEGYLLTGGMMLWFRDQYLNSLEELTHPWFSPVLYPDLSGLPPAYIATAQYDPLRDVGKLYAEALNKAGVKVEIENFEDLIHGFAGFYSLSPGATKALVRIAEKLRDALA

SEQ ID NO: 27 - DNA, 930 bp, synthetic construct
  misc_feature 1..930: note = Description of Artificial Sequence: Syntheticpolynucleotide sequence encoding a codon optimizedcarboxyesterase enzyme
  source 1..930: mol_type = other DNA
atgccattagatcctgtgattcaacaagtcctcgatcaactgaaccgtatgccagcccctgactacaagcacttaagcgctcaacagtttcgttcacagcagtcactgtttccaccagttaagaaagaaccggtcgcagaagttcgcgaattcgacatggatctgccgatgcgtaccctgaaagtccgtatgtaccgtccggaaggtgttgaaccaccatatccagcactggtttactaccatggtggcggttgggttgttggtgacctggaaacgcatgatccggtgtgtcgtgtgttggcgaaatggggacgcgcagtggtgtttagcgttgactaccgtctggcaccagaacacaagtttccagcggcagttgaagacgcgtatgatgcactgcaatggattgcagaacgtgcagccgatttccatcttgatccagcacgcattgcagttggcggcgattcagcaggcggcaacctggcggccgtgactagtattctggcgaaagaacgtggtggtccagcaattgcgtttcaactgctgatctatccctccactggttatgatccagcacatccaccagcaagtatccttgagaatgcggagggttacctgttaacccatggcatgatgctgtggtttcgtgaccagtacctgaacagccttgaggaactgactcacccatggtttagtccagtgctgtacccggatcttagcggtttaccaccggcgtacattgcaaccgcacagtacgatcccctgcgcgatgtcggcaaactttacgctgaagccctgaacaaagcgggcgttaaagtggagatcgagaacttcgaggatctgattcatggcttcgcggggttctattctctgagcccaggcgcaaccagagcactggtacgtattgccgagaaactgcgcgatgcgttggcg

SEQ ID NO: 28 - protein, 310 aa, synthetic construct
  REGION 1..310: note = Description of Artificial Sequence: Syntheticpolypeptide sequence of a codon optimizedcarboxyesterase enzyme
MPLDPVIQQVLDQLNRMPAPDYKHLSAQQFRSQQSLFPPVKKEPVAEVREFDMDLPMRTLKVRMYRPEGVEPPYPALVYYHGGGWVVGDLETHDPVCRVLAKWGRAVVFSVDYRLAPEHKFPAAVEDAYDALQWIAERAADFHLDPARIAVGGDSAGGNLAAVTSILAKERGGPAIAFQLLIYPSTGYDPAHPPASILENAEGYLLTHGMMLWFRDQYLNSLEELTHPWFSPVLYPDLSGLPPAYIATAQYDPLRDVGKLYAEALNKAGVKVEIENFEDLIHGFAGFYSLSPGATRALVRIAEKLRDALA

SEQ ID NO: 29 - DNA, 930 bp, synthetic construct
  misc_feature 1..930: note = Description of Artificial Sequence: Syntheticpolynucleotide sequence encoding a codon optimizedcarboxyesterase enzyme
  source 1..930: mol_type = other DNA
atgccattagatcctgtgattcaacaagtcctcgatcaactgaaccgtatgccagcccctgactacaagcacttaagcgctcaacagtttcgttcacagcaatcactgtttccgccagttaagaaagaaccggtcgcagaagttcgcgaattcgacatggatctgccgggccgtaccctgaaagtccgtatgtaccgtccggaaggtgttgaaccaccatatccagcactggtttactaccatggtggcggttgggttgttggtgacctggaaacgcatgatccggtgtgtcgtgtgttggcgaaagatggacgcgcagtggtgtttagcgttgactaccgtctggcaccagaacacaagtttccagcggcagttgaagacgcgtatgatgcactgcaatggattgcagaacgtgccgccgatttccatcttgatccagcacgcattgcagttggcggcgattcagcaggcggcaacctggcggccgtgactagtattctggcgaaagaacgtggtggtccagcaattgcgtttcaactgctgatctatccctccactggttatgatccagcacatccaccagcaagtatccttgagaatgcggagggttacctgttaaccggaggcatgatgctgtggtttcgtgaccagtacctgaacagccttgaggaactgactcacccatggtttagtccagtgctgtacccggatcttagcggtttaccaccggcgtacattgcaaccgcacagtacgatcccctgcgcgatgtcggcaaactttacgctgaagccctgaacaaagcgggcgttaaagtggagatcgagaacttcgaggatctgattcatggcttcgcggggttctattctctgagcccaggcgcaaccaaagcactggtacgtattgccgagaaactgcgcgatgcgttggcg

SEQ ID NO: 30 - protein, 310 aa, synthetic construct
  REGION 1..310: note = Description of Artificial Sequence: Syntheticpolypeptide sequence of a codon optimizedcarboxyesterase enzyme
MPLDPVIQQVLDQLNRMPAPDYKHLSAQQFRSQQSLFPPVKKEPVAEVREFDMDLPGRTLKVRMYRPEGVEPPYPALVYYHGGGWVVGDLETHDPVCRVLAKDGRAVVFSVDYRLAPEHKFPAAVEDAYDALQWIAERAADFHLDPARIAVGGDSAGGNLAAVTSILAKERGGPAIAFQLLIYPSTGYDPAHPPASILENAEGYLLTGGMMLWFRDQYLNSLEELTHPWFSPVLYPDLSGLPPAYIATAQYDPLRDVGKLYAEALNKAGVKVEIENFEDLIHGFAGFYSLSPGATKALVRIAEKLRDALA

SEQ ID NO: 31 - DNA, 930 bp, synthetic construct
  misc_feature 1..930: note = Description of Artificial Sequence: Syntheticpolynucleotide sequence encoding a codon optimizedcarboxyesterase enzyme
  source 1..930: mol_type = other DNA
atgccattagatcctgtgattcaacaagtcctcgatcaactgaaccgtatgccagcccctgactacaagcacttaagcgctcaacagtttcgttcacagcaatcactgtttccgccagttaagaaagaaccggtcgcagaagttcgcgaattcgacatggatctgccgggccgtaccctgaaagtccgtatgtaccgtccggaaggtgttgaaccaccatatccagcactggtttactaccatggtggcggttgggttgttggtgacctggaaacgcatgatccggtgtgtcgtgtgttggcgaaatggggacgcgcagtggtgtttagcgttgactaccgtctggcaccagaacacaagtttccagcggcagttgaagacgcgtatgatgcactgcaatggattgcagaacgtgccgccgatttccatcttgatccagcacgcattgcagttggcggcgattcagcaggcggcaacctggcggccgtgactagtattctggcgaaagaacgtggtggtccagcaattgcgtttcaactgctgatctatccctccactggttatgatccagcacatccaccagcaagtatcattgagaatgcggagggttacctgttaaccggtggcatgatgctgtggtttcgtgaccagtacctgaacagccttgaggaactgactcacccatggtttagtccagtgctgtacccggatcttagcggtttaccaccggcgtacattgcaaccgcacagtacgatcccctgcgcgatgtcggcaaactttacgctgaagccctgaacaaagcgggcgttaaagtggagatcgagaacttcgaggatctgattcatggcttcgcggggttctattctctgagcccaggcgcaaccaaagcactggtacgtattgccgagaaactgcgcgatgcgttggcg

SEQ ID NO: 32 - protein, 310 aa, synthetic construct
  REGION 1..310: note = Description of Artificial Sequence: Syntheticpolypeptide sequence of a codon optimizedcarboxyesterase enzyme
MPLDPVIQQVLDQLNRMPAPDYKHLSAQQFRSQQSLFPPVKKEPVAEVREFDMDLPGRTLKVRMYRPEGVEPPYPALVYYHGGGWVVGDLETHDPVCRVLAKWGRAVVFSVDYRLAPEHKFPAAVEDAYDALQWIAERAADFHLDPARIAVGGDSAGGNLAAVTSILAKERGGPAIAFQLLIYPSTGYDPAHPPASIIENAEGYLLTGGMMLWFRDQYLNSLEELTHPWFSPVLYPDLSGLPPAYIATAQYDPLRDVGKLYAEALNKAGVKVEIENFEDLIHGFAGFYSLSPGATKALVRIAEKLRDALA

SEQ ID NO: 33 - DNA, 930 bp, synthetic construct
  misc_feature 1..930: note = Description of Artificial Sequence: Syntheticpolynucleotide sequence encoding a codon optimizedcarboxyesterase enzyme
  source 1..930: mol_type = other DNA
atgccattagatcctgtgattcaacaagtcctcgatcaactgaaccgtatgccagcccctgactacaagcacttaagcgctcaacagtttcgttcacagcaatcactgtttccaccagttaagaaagaaccggtcgcagaagttcgcgaattcgacatggatctgccgggccgtaccctgaaagtccgtatgtaccgtccggaaggtgttgaaccaccatatccagcactggtttactaccatggtggcggttgggttgttggtgacctggaaacgcatgatccggtgtgtcgtgtgttggcgaaatggggacgcgcagtggtgtttagcgttgactaccgtctggcaccagaacacaagtttccagcggcagttgaagacgcgtatgatgcactgcaatggattgcagaacgtgccgccgatttccatcttgatccagcacgcattgcagttggcggcgattcagcaggcggcaacctggcggccgtgactagtattctggcgaaagaacgtggtggtccagcaattgcgtttcaactgctgatctatccctccactggttatgatccagcacatccaccagcaagtatccttgagaatgcggagggttacctgttaaccggtggcatgatgctgtggtttcgtgaccagtacctgaacagccttgaggaactgactcacccatggtttagtccagtgctgtacccggatcttagcggtttaccaccggcgtacattgcaaccgcacagtacgatcccctgcgcgatgtcggcaaactttacgctgaagccctgaacaaagcgggcgttgatgtggagatcgagaacttcgaggatctgattcatggcttcgcggggttctattctctgagcccaggcgcaaccaaagcactggtacgtattgccgagaaactgcgcgatgcgttggcg

SEQ ID NO: 34 - protein, 310 aa, synthetic construct
  REGION 1..310: note = Description of Artificial Sequence: Syntheticpolypeptide sequence of a codon optimizedcarboxyesterase enzyme
MPLDPVIQQVLDQLNRMPAPDYKHLSAQQFRSQQSLFPPVKKEPVAEVREFDMDLPGRTLKVRMYRPEGVEPPYPALVYYHGGGWVVGDLETHDPVCRVLAKWGRAVVFSVDYRLAPEHKFPAAVEDAYDALQWIAERAADFHLDPARIAVGGDSAGGNLAAVTSILAKERGGPAIAFQLLIYPSTGYDPAHPPASILENAEGYLLTGGMMLWFRDQYLNSLEELTHPWFSPVLYPDLSGLPPAYIATAQYDPLRDVGKLYAEALNKAGVDVEIENFEDLIHGFAGFYSLSPGATKALVRIAEKLRDALA

SEQ ID NO: 35 - DNA, 930 bp, synthetic construct
  misc_feature 1..930: note = Description of Artificial Sequence: Syntheticpolynucleotide sequence encoding a codon optimizedcarboxyesterase enzyme
  source 1..930: mol_type = other DNA
atgccattagatcctgtgattcaatatgtcctcgatcaactgaaccgtatgccagcccctgactacaagcacttaagcgctcaacagtttcgttcacagcaacacctgaccccaccagttaagaaagaaccggtcgcagaagttcgcgaattcgacatggatctgccgggccgtaccctgaaagtccgtatgtaccgcccggaaggtgttgaaccaccatatccagcactggtttactaccatggtggcggttgggttgttggtgacctggaaacgcatgatccggtgtgtcgtgtgttggcgaaatggggacgcgcagtggtgtttagcgttgactaccgtctggcaccagaacacaagtttccagcggcagttgaagacgcgtatgatgcactgcaatggattgcagaacgtgcagccgatttccatcttgatccagcacgcattgcagttggcggcgattcagcaggcggcaacctggcggccgtgactagtattctggcgaaagaacgtggtggtccagcaattgcgtttcaactgctgatctatccctttactggttatgatccagcacatccaccagcaagtatccttgagaatgcggagggttacctgttaaccggaggcatgatgctgtggtttcgtgaccagtacctgaacagccttgaggaactgactcacccatggtttagtccagtgctgtacccggatcttagcggtttaccaccggcgtacattgcaaccgcacagtacgatcccctgcgcgatgtcggcaaactttacgctgaagccctgaacaaagcgggcgttaaggtggagatcgagaacttcgaggatctgattcatggcttcgcgcagttctattctctgagcccaggcgcaaccaaagcactggtacgtattgccgagaaactgcgcgatgcgttggcg

SEQ ID NO: 36 - protein, 310 aa, synthetic construct
  REGION 1..310: note = Description of Artificial Sequence: Syntheticpolypeptide sequence of a codon optimizedcarboxyesterase enzyme
MPLDPVIQYVLDQLNRMPAPDYKHLSAQQFRSQQHLTPPVKKEPVAEVREFDMDLPGRTLKVRMYRPEGVEPPYPALVYYHGGGWVVGDLETHDPVCRVLAKWGRAVVFSVDYRLAPEHKFPAAVEDAYDALQWIAERAADFHLDPARIAVGGDSAGGNLAAVTSILAKERGGPAIAFQLLIYPFTGYDPAHPPASILENAEGYLLTGGMMLWFRDQYLNSLEELTHPWFSPVLYPDLSGLPPAYIATAQYDPLRDVGKLYAEALNKAGVKVEIENFEDLIHGFAQFYSLSPGATKALVRIAEKLRDALA

SEQ ID NO: 37 - DNA, 930 bp, synthetic construct
  misc_feature 1..930: note = Description of Artificial Sequence: Syntheticpolynucleotide sequence encoding a codon optimizedcarboxyesterase enzyme
  source 1..930: mol_type = other DNA
atgccattagatcctgtgattcaacaagtcctcgatcaactgaaccgtatgccagcccctgactacaagcacttaagcgctcaacagtttcgttcacagcaaagcctgtttccaccagttaagaaagaaccggtcgcagaactgcgcgaattcgacatggatctgccgggccgtaccctgaaagtccgtatgtaccgcccggaaggtgttgaaccaccatatccagcactggtttactaccatggtggcggttgggttgttggtgacctggaaacgcatgatccggtgtgtcgtgtgttggcgaaagatggacgcgcagtggtgtttagcgttgactaccgtctggcaccagaacacaagtttccagcggcagttgaagacgcgtatgatgcactgcaatggattgcagaacgtgcagccgatttccatcttgatccagcacgcattgcagttggcggcgattcagcaggcggcaacctggcggccgtgactagtattctggcgaaagaacgtggtggtccagcaattgcgtttcaactgctgatctatccctttactggttatgatccagcacatccaccagcaagtatccttgagaatgcggagggttacctgttaaccggaggcatgatgctgtggtttcgtaaccagtacctgaacagccttgaggaactgactcacccatggtttagtccagtgctgtacccggatcttagcggtttaccaccggcgtacattgcaaccgcacagtacgatcccctgcgcgatgtcggcaaactttacgctgaagccctgaacaaagcgggcgttaaggtggagatcgagaacttcgaggatctgattcatggcttcgcgcagttctattctctgagcccaggcgcaaccaaagcactggtacgtattgccgagaaactgcgcgatgcgttggcg

SEQ ID NO: 38 - protein, 310 aa, synthetic construct
  REGION 1..310: note = Description of Artificial Sequence: Syntheticpolypeptide sequence of a codon optimizedcarboxyesterase enzyme
MPLDPVIQQVLDQLNRMPAPDYKHLSAQQFRSQQSLFPPVKKEPVAELREFDMDLPGRTLKVRMYRPEGVEPPYPALVYYHGGGWVVGDLETHDPVCRVLAKDGRAVVFSVDYRLAPEHKFPAAVEDAYDALQWIAERAADFHLDPARIAVGGDSAGGNLAAVTSILAKERGGPAIAFQLLIYPFTGYDPAHPPASILENAEGYLLTGGMMLWFRNQYLNSLEELTHPWFSPVLYPDLSGLPPAYIATAQYDPLRDVGKLYAEALNKAGVKVEIENFEDLIHGFAQFYSLSPGATKALVRIAEKLRDALA

SEQ ID NO: 39 - DNA, 930 bp, synthetic construct
  misc_feature 1..930: note = Description of Artificial Sequence: Syntheticpolynucleotide sequence encoding a codon optimizedcarboxyesterase enzyme
  source 1..930: mol_type = other DNA
atgccattagatcctgtgattcaatatgtcctcgatcaactgaaccgtatgccacgtcctgactacaagcacttaagcgctcaacagtttcgttcacagaaccacctgtttccaccagttaagaaagaaccggtcgcagaagttcgcgaattcgacatggatctgccgggccgtaccctgaaagtccgtatgtaccgcccggaaggtgttgaaccaccatatccagcactggtttactaccatggtggcggttgggttgcgggtgacctggaaacgcatgatccggtgtgtcgtgtgttggcgaaagatggacgcgcagtggtgtttagcgttgactaccgtctggcaccagaacacaagtttccagcggcagttgaagacgcgtatgatgcactgcaatggattgcagaacgtgcagccgatttccatcttgatccagcacgcattgcagttggcggcgattcagcaggcggcaacctggcggccgtgactagtattctggcgaaagaacgtggtggtccagcaattgcgtttcaactgctgatctatccctttactggttatgatccagcacatccaccagcaagtatccttgagaatgcggagggttacctgttaaccggaggcatgatgctgtggtttcgtgaccagtacctgaacagccttgaggaactgactcacccatggtttagtccagtgctgtacccggatcttagcggtttaccaccggcgtacattgcaaccgcacagtacgatcccctgcgcgatgtcggcaaactttacgctgaagccctgaacaaagcgggcgttgatgtggagatcgagaacttcgaggatctgattcatggcttcgcgcagttctattctctgagcccaggcgcaacccgtgcactggtacgtattgccgagaaactgcgcgatgcgttggcg

SEQ ID NO: 40 - protein, 310 aa, synthetic construct
  REGION 1..310: note = Description of Artificial Sequence: Syntheticpolypeptide sequence of a codon optimizedcarboxyesterase enzyme
MPLDPVIQYVLDQLNRMPRPDYKHLSAQQFRSQNHLFPPVKKEPVAEVREFDMDLPGRTLKVRMYRPEGVEPPYPALVYYHGGGWVAGDLETHDPVCRVLAKDGRAVVFSVDYRLAPEHKFPAAVEDAYDALQWIAERAADFHLDPARIAVGGDSAGGNLAAVTSILAKERGGPAIAFQLLIYPFTGYDPAHPPASILENAEGYLLTGGMMLWFRDQYLNSLEELTHPWFSPVLYPDLSGLPPAYIATAQYDPLRDVGKLYAEALNKAGVDVEIENFEDLIHGFAQFYSLSPGATRALVRIAEKLRDALA

SEQ ID NO: 41 - DNA, 930 bp, synthetic construct
  misc_feature 1..930: note = Description of Artificial Sequence: Syntheticpolynucleotide sequence encoding a codon optimizedcarboxyesterase enzyme
  source 1..930: mol_type = other DNA
atgccattagatcctgtgattcaatatgtcctcgatcaactgaaccgtatgccagcccctgactacaagcacttaagcgctcaacagtttcgttcacaggaacacctgtttccaccagttaagaaagaaccggtcgcagaagttcgcgaattcgacatggatctgccgggccgtaccctgaaagtccgtatgtaccgcccggaaggtgttgaaccaccatatccagcactggtttactaccatggtggcggttgggttgcgggtgacctggaaacgcatgatccggtgtgtcgtgtgttggcgaaagatggacgcgcagtggtgtttagcgttgactaccgtctggcaccagaacacaagtttccagcggcagttgaagacgcgtatgatgcactgcaatggattgcagaacgtgcagccgatttccatcttgatccagcacgcattgcagttggcggcgattcagcaggcggcaacctggcggccgtgactagtattctggcgaaagaacgtggtggtccagcaattgcgtttcaactgctgatctatccctttactggttatgatccagcacatccaccagcaagtatccttgagaatgcggagggttacctgttaaccggaggcatgatgctgtggtttcgtgaccagtacctgaacagccttgaggaactgactcacccatggtttagtccagtgctgtacccggatcttagcggtttaccaccggcgtacattgcaaccgcacagtacgatcccctgcgcgatgtcggcaaactttacgctgaagccctgaacaaagcgggcgttgatgtggagatcgagaacttcgaggatctgattcatggcttcgcgcagttctattctctgagcccaggcgcaaccaaagcactggtacgtattgccgagaaactgcgcgatgcgttggcg

SEQ ID NO: 42 - protein, 310 aa, synthetic construct
  REGION 1..310: note = Description of Artificial Sequence: Syntheticpolypeptide sequence of a codon optimizedcarboxyesterase enzyme
MPLDPVIQYVLDQLNRMPAPDYKHLSAQQFRSQEHLFPPVKKEPVAEVREFDMDLPGRTLKVRMYRPEGVEPPYPALVYYHGGGWVAGDLETHDPVCRVLAKDGRAVVFSVDYRLAPEHKFPAAVEDAYDALQWIAERAADFHLDPARIAVGGDSAGGNLAAVTSILAKERGGPAIAFQLLIYPFTGYDPAHPPASILENAEGYLLTGGMMLWFRDQYLNSLEELTHPWFSPVLYPDLSGLPPAYIATAQYDPLRDVGKLYAEALNKAGVDVEIENFEDLIHGFAQFYSLSPGATKALVRIAEKLRDALA

SEQ ID NO: 43 - DNA, 930 bp, synthetic construct
  misc_feature 1..930: note = Description of Artificial Sequence: Syntheticpolynucleotide sequence encoding a codon optimizedcarboxyesterase enzyme
  source 1..930: mol_type = other DNA
atgccattagatcctgtgattcaatatgtcctcgatcaactgaaccgtatgccacgtcctgactacaagcacttaagcgctcaacagtttcgttcacaggaacacctgtttccaccagttaagaaagaaccggtcgtggaagttcgcgaattcgacatggatctgccgggccgtaccctgaaagtccgtatgtaccgcccggaaggtgttgaaccaccatatccagcactggtttactaccatggtggcggttgggttgcgggtgacctggaaacgcatgatccggtgtgtcgtgtgttggcgaaagatggacgcgcagtggtgtttagcgttgactaccgtctggcaccagaacacaagtttccagcggcagttgaagacgcgtatgatgcactgcaatggattgcagaacgtgcagccgatttccatcttgatccagcacgcattgcagttggcggcgattcagcaggcggcaacctggcggccgtgactagtattctggcgaaagaacgtggtggtccagcaattgcgtttcaactgctgatctatccctttactggttatgatccagcacatccaccagcaagtatccttgagaatgcggagggttacctgttaaccggaggcatgatgctgtggtttcgtgaccagtacctgaacagccttgaggaactgactcacccatggtttagtccagtgctgtacccggatcttagcggtttaccaccggcgtacattgcaaccgcacagtacgatcccctgcgcgatgtcggcaaactttacgctgaagccctgaacaaagcgggcgttgatgtggagatcgagaacttccaggatctgattcatggcttcgcgcagttctattctctgagcccaggcgcaacccgtgcactggtacgtattgccgagaaactgcgcgatgcgttggcg

SEQ ID NO: 44 - protein, 310 aa, synthetic construct
  REGION 1..310: note = Description of Artificial Sequence: Syntheticpolypeptide sequence of a codon optimizedcarboxyesterase enzyme
MPLDPVIQYVLDQLNRMPRPDYKHLSAQQFRSQEHLFPPVKKEPVVEVREFDMDLPGRTLKVRMYRPEGVEPPYPALVYYHGGGWVAGDLETHDPVCRVLAKDGRAVVFSVDYRLAPEHKFPAAVEDAYDALQWIAERAADFHLDPARIAVGGDSAGGNLAAVTSILAKERGGPAIAFQLLIYPFTGYDPAHPPASILENAEGYLLTGGMMLWFRDQYLNSLEELTHPWFSPVLYPDLSGLPPAYIATAQYDPLRDVGKLYAEALNKAGVDVEIENFQDLIHGFAQFYSLSPGATRALVRIAEKLRDALA

SEQ ID NO: 45 - DNA, 930 bp, synthetic construct
  misc_feature 1..930: note = Description of Artificial Sequence: Syntheticpolynucleotide sequence encoding a codon optimizedcarboxyesterase enzyme
  source 1..930: mol_type = other DNA
atgccattagatcctgtgattcaatatgtcctcgatcaactgaaccgtatgccagcccctgactacaagcacttaagcgctcaacagtttcgttcacagaaccacctgtttccaccagttaagaaagaaccggtcgtggaagttcgcgaattcgacatggatctgccgggccgtaccctgaaagtccgtatgtaccgcccggaaggtgttgaaccaccatatccagcactggtttactaccatggtggcggttgggttgcgggtgacctggaaacgcatgatccggtgtgtcgtgtgttggcgaaagatggacgcgcagtggtgtttagcgttgactaccgtctggcaccagaacacaagtttccagcggcagttgaagacgcgtatgatgcactgcaatggattgcagaacgtgcagccgatttccatcttgatccagcacgcattgcagttggcggcgattcagcaggcggcaacctggcggccgtgactagtattctggcgaaagaacgtggtggtccagcaattgcgtttcaactgctgatctatccctttactggttatgatccagcacatccaccagcaagtatccttgagaatgcggagggttacctgttaaccggaggcatgatgctgtggtttcgtgaccagtacctgaacagccttgaggaactgactcacccatggtttagtccagtgctgtacccggatcttagcggtttaccaccggcgtacattgcaaccgcacagtacgatcccctgcgcgatgtcggcaaactttacgctgaagccctgaacaaagcgggcgttaaggtggagatcgagaacttccaggatctgattcatggcttcgcgcagttctattctctgagcccaggcgcaacccgtgcactggtacgtattgccgagaaactgcgcgatgcgttggcg

SEQ ID NO: 46 - protein, 310 aa, synthetic construct
  REGION 1..310: note = Description of Artificial Sequence: Syntheticpolypeptide sequence of a codon optimizedcarboxyesterase enzyme
MPLDPVIQYVLDQLNRMPAPDYKHLSAQQFRSQNHLFPPVKKEPVVEVREFDMDLPGRTLKVRMYRPEGVEPPYPALVYYHGGGWVAGDLETHDPVCRVLAKDGRAVVFSVDYRLAPEHKFPAAVEDAYDALQWIAERAADFHLDPARIAVGGDSAGGNLAAVTSILAKERGGPAIAFQLLIYPFTGYDPAHPPASILENAEGYLLTGGMMLWFRDQYLNSLEELTHPWFSPVLYPDLSGLPPAYIATAQYDPLRDVGKLYAEALNKAGVKVEIENFQDLIHGFAQFYSLSPGATRALVRIAEKLRDALA

SEQ ID NO: 47 - DNA, 930 bp, synthetic construct
  misc_feature 1..930: note = Description of Artificial Sequence: Syntheticpolynucleotide sequence encoding a codon optimizedcarboxyesterase enzyme
  source 1..930: mol_type = other DNA
atgccattagatcctgtgattcaacaagtcctcgatcaactgaaccgtatgccagcccctgactacaagcacttaagcgctcaacagtttcgttcacagcaacacctgtttccaccagttaagaaagaaccggtcgcagaagttcgcgaattcgacatggatctgccgggccgtaccctgaaagtccgtatgtacgtgccggaaggtgttgaaccaccatatccagcactggtttactaccatggtggcggttgggttgttggtgacctggaaacgcatgatccggtgtgtcgtgtgttggcgaaagatggacgcgcagtggtgtttagcgttgactaccgtctggcaccagaacacaagtttccagcggcagttgaagacgcgtatgatgcactgcaatggattgcagaacgtgcagccgatttccatcttgatccagcacgcattgcagttggcggcgattcagcaggcggcaacctggcggccgtgactagtattctggcgaaagaacgtggtggtccagcaattgcgtttcaactgctgatctatccctttactggttatgattatgcacatccaccagcaagtatccttgagaatgcggagggttacctgttagaaggaggcatgatgctgtggtttcgtgaccagtacctgaacagccttgaggaactgactcacccatggtttagtccagtgctgtacccggatcttagcggtttaccaccggcgtacattgcaaccgcacagtacgatcccctgcgcgatgtcggcaaactttacgctaccgccctgaacaaagcgggcgttaaggtggagatcgagaacttcgaggatctgattcatggcttcgcgcagttctattctctgagcccaggcgcaaccaaagcactggtacgtattgccgagaaactgcgcgatgcgttggcg

SEQ ID NO: 48 - protein, 310 aa, synthetic construct
  REGION 1..310: note = Description of Artificial Sequence: Syntheticpolypeptide sequence of a codon optimizedcarboxyesterase enzyme
MPLDPVIQQVLDQLNRMPAPDYKHLSAQQFRSQQHLFPPVKKEPVAEVREFDMDLPGRTLKVRMYVPEGVEPPYPALVYYHGGGWVVGDLETHDPVCRVLAKDGRAVVFSVDYRLAPEHKFPAAVEDAYDALQWIAERAADFHLDPARIAVGGDSAGGNLAAVTSILAKERGGPAIAFQLLIYPFTGYDYAHPPASILENAEGYLLEGGMMLWFRDQYLNSLEELTHPWFSPVLYPDLSGLPPAYIATAQYDPLRDVGKLYATALNKAGVKVEIENFEDLIHGFAQFYSLSPGATKALVRIAEKLRDALA

SEQ ID NO: 49 - DNA, 930 bp, synthetic construct
  misc_feature 1..930: note = Description of Artificial Sequence: Syntheticpolynucleotide sequence encoding a codon optimizedcarboxyesterase enzyme
  source 1..930: mol_type = other DNA
atgccattagatcctgtgattcaatatgtcctcgatcaactgaaccgtatgccagcccctgactacaagcacttaagcgctcaacagtttcgttcacaggaacacctgtttccaccagttaagaaagaaccggtcgtggaagttcgcgaattcgacatggatctgccgggccgtaccctgaaagtccgtatgtaccgcccggaaggtgttgaaccaccatatccagcactggtttactaccatggtggcggttgggttgcgggtgacctggaaacgcatgatccggtgtgtcgtgtgttggcgaaagatggacgcgcagtggtgtttagcgttgactaccgtctggcaccagaacacaagtttccagcggcagttgaagacgcgtatgatgcactgcaatggattgcagaacgtcgtgccgatttccatcttgatccagcacgcattgcagttggcggcgattcagcaggcggcaacctggcggccgtgactagtattctggcgaaagaacgtggtggtccagcaattgcgtttcaactgctgatctatccctttactggttatgatccagcacatccaccagcaagtatccttgagaatgcggagggttacctgttaaccggaggcatgatgctgtggtttcgtgaccagtacctgaacagccttgaggaactgactcacccatggtttagtccagtgctgtacccggatcttagcggtttaccaccggcgtacattgcaaccgcacagtacgatcccctgcgcgatgtcggcaaactttacgctgaagccctgaacaaagcgggcgttaaggtggagatcgagaacttcgaggatctgattcatggcttcgcgcagttctattctctgagcccaggcgcaaccaaagcactggtacgtattgccgagaaactgcgcgatgcgttggcg

SEQ ID NO: 50 - protein, 310 aa, synthetic construct
  REGION 1..310: note = Description of Artificial Sequence: Syntheticpolypeptide sequence of a codon optimizedcarboxyesterase enzyme
MPLDPVIQYVLDQLNRMPAPDYKHLSAQQFRSQEHLFPPVKKEPVVEVREFDMDLPGRTLKVRMYRPEGVEPPYPALVYYHGGGWVAGDLETHDPVCRVLAKDGRAVVFSVDYRLAPEHKFPAAVEDAYDALQWIAERRADFHLDPARIAVGGDSAGGNLAAVTSILAKERGGPAIAFQLLIYPFTGYDPAHPPASILENAEGYLLTGGMMLWFRDQYLNSLEELTHPWFSPVLYPDLSGLPPAYIATAQYDPLRDVGKLYAEALNKAGVKVEIENFEDLIHGFAQFYSLSPGATKALVRIAEKLRDALA

SEQ ID NO: 51 - DNA, 930 bp, synthetic construct
  misc_feature 1..930: note = Description of Artificial Sequence: Syntheticpolynucleotide sequence encoding a codon optimizedcarboxyesterase enzyme
  source 1..930: mol_type = other DNA
atgccattagatcctgtgattcaatatgtcctcgatcaactgaaccgtatgccagcccctgactacaagcacttaagcgctcaacagtttcgttcacagaaccacctgtttccaccagttaagaaagaaccggtcgcagaagttcgcgaattcgacatggatctgccgggccgtaccctgaaagtccgtatgtaccgcccggaaggtgttgaaccaccatatccagcactggtttactaccatggtggcggttgggttgcgggtgacctggaaacgcatgatccggtgtgtcgtgtgttggcgaaagatggacgcgcagtggtgtttagcgttgactaccgtctggcaccagaacacaagtttccagcggcagttgaagacgcgtatgatgcactgcaatggattgcagaacgtgcagccgatttccatcttgatccagcacgcattgcagttggcggcgattcagcaggcggcaacctggcggccgtgactagtattctggcgaaagaacgtggtggtccagcaattgcgtttcaactgctgatctatccctttactggttatgatccagcacatccaccagcaagtatccttgagaatgcggagggttacctgttaaccggaggcatgatgctgtggtttcgtgaccagtacctgaacagccttgaggaactgactcacccatggtttagtccagtgctgtacccggatcttagcggtttaccaccggcgtacattgcaaccgcacagtacgatcccctgcgcgatgtcggcaaactttacgctgaagccctgaacaaagcgggcgttaaggtggagatcgagaacttcgaggatctgattcatggcttcgcgcagttctattctctgagcccaggcgcaacccgtgcactggtacgtattgccgagaaactgcgcgatgcgttggcg

SEQ ID NO: 52 - protein, 310 aa, synthetic construct
  REGION 1..310: note = Description of Artificial Sequence: Syntheticpolypeptide sequence of a codon optimizedcarboxyesterase enzyme
MPLDPVIQYVLDQLNRMPAPDYKHLSAQQFRSQNHLFPPVKKEPVAEVREFDMDLPGRTLKVRMYRPEGVEPPYPALVYYHGGGWVAGDLETHDPVCRVLAKDGRAVVFSVDYRLAPEHKFPAAVEDAYDALQWIAERAADFHLDPARIAVGGDSAGGNLAAVTSILAKERGGPAIAFQLLIYPFTGYDPAHPPASILENAEGYLLTGGMMLWFRDQYLNSLEELTHPWFSPVLYPDLSGLPPAYIATAQYDPLRDVGKLYAEALNKAGVKVEIENFEDLIHGFAQFYSLSPGATRALVRIAEKLRDALA

SEQ ID NO: 53 - DNA, 930 bp, synthetic construct
  misc_feature 1..930: note = Description of Artificial Sequence: Syntheticpolynucleotide sequence encoding a codon optimizedcarboxyesterase enzyme
  source 1..930: mol_type = other DNA
atgccattagatcctgtgattcaatatgtcctcgatcaactgaaccgtatgccagcccctgactacaagcacttaagcgctcaacagtttcgttcacagcaacacctgtttccaccagttaagaaagaaccggtcgcagaagttcgcgaattcgacatggatctgccgggccgtaccctgaaagtccgtatgtaccgcccggaaggtgttgaaccaccatatccagcactggtttactaccatggtggcggttgggttgcgggtgacctggaaacgcatgatccggtgtgtcgtgtgttggcgaaagatggacgcgcagtggtgtttagcgttgactaccgtctggcaccagaacacaagtttccagcggcagttgaagacgcgtatgatgcactgcaatggattgcagaacgtgcagccgatttccatcttgatccagcacgcattgcagttggcggcgattcagcaggcggcaacctggcggccgtgactagtattctggcgaaagaacgtggtggtccagcaattgcgtttcaactgctgatctatccctttactggttatgatccagcacatccaccagcaagtatccttgagaatgcggagggttacctgttaaccggaggcatgatgctgtggtttcgtgaccagtacctgaacagccttgaggaactgactcacccatggtttagtccagtgctgtacccggatcttagcggtttaccaccggcgtacattgcaaccgcacagtacgatcccctgcgcgatgtcggcaaactttacgctgaagccctgaacaaagcgggcgttaaggtggagatcgagaacttcgaggatctgattcatggcttcgcgcagttctattctctgagcccaggcgcaaccaaagcactggtacgtattgccgagaaactgcgcgatgcgttggcg

SEQ ID NO: 54 - protein, 310 aa, synthetic construct
  REGION 1..310: note = Description of Artificial Sequence: Syntheticpolypeptide sequence of a codon optimizedcarboxyesterase enzyme
MPLDPVIQYVLDQLNRMPAPDYKHLSAQQFRSQQHLFPPVKKEPVAEVREFDMDLPGRTLKVRMYRPEGVEPPYPALVYYHGGGWVAGDLETHDPVCRVLAKDGRAVVFSVDYRLAPEHKFPAAVEDAYDALQWIAERAADFHLDPARIAVGGDSAGGNLAAVTSILAKERGGPAIAFQLLIYPFTGYDPAHPPASILENAEGYLLTGGMMLWFRDQYLNSLEELTHPWFSPVLYPDLSGLPPAYIATAQYDPLRDVGKLYAEALNKAGVKVEIENFEDLIHGFAQFYSLSPGATKALVRIAEKLRDALA

SEQ ID NO: 55 - DNA, 930 bp, synthetic construct
  misc_feature 1..930: note = Description of Artificial Sequence: Syntheticpolynucleotide sequence encoding a codon optimizedcarboxyesterase enzyme
  source 1..930: mol_type = other DNA
atgccattagatcctgtgattcaatatgtcctcgatcaactgaaccgtatgccagcccctgactacaagcacttaagcgctcaacagtttcgttcacagcaacacctgtttccaccagttaagaaagaaccggtcgcagaagttcgcgaattcgacatggatctgccgggccgtaccctgaaagtccgtatgtaccgcccggaaggtgttgaaccaccatatccagcactggtttactaccatggtggcggttgggttgcgggtgacctggaaacgcatgatccggtgtgtcgtgtgttggcgaaagatggacgcgcagtggtgtttagcgttgactaccgtctggcaccagaacacaagtttccagcggcagttgaagacgcgtatgatgcactgcaatggattgcagaacgtgcagccgatttccatcttgatccagcacgcattgcagttggcggcgattcagcaggcggcaacctggcggccgtgactagtattctggcgaaagaacgtggtggtccagcaattgcgtttcaactgctgatctatccctttactggttatgatccagcacatccaccagcaagtatccttgagaatgcggagggttacctgttaaccggaggcatgatgctgtggtttcgtgaccagtacctgaacagccttgaggaactgactcacccatggtttagtccagtgctgtacccggatcttagcggtttaccaccggcgtacattgcaaccgcacagtacgatcccctgcgcgatgtcggcaaactttacgctgaagccctgaacaaagcgggcgttaaggtggagatcgagaacttcgaggatctgattcatggcttcgcgagtttctattctctgagcccaggcgcaaccaaagcactggtacgtattgccgagaaactgcgcgatgcgttggcg

SEQ ID NO: 56 - protein, 310 aa, synthetic construct
  REGION 1..310: note = Description of Artificial Sequence: Syntheticpolypeptide sequence of a codon optimizedcarboxyesterase enzyme
MPLDPVIQYVLDQLNRMPAPDYKHLSAQQFRSQQHLFPPVKKEPVAEVREFDMDLPGRTLKVRMYRPEGVEPPYPALVYYHGGGWVAGDLETHDPVCRVLAKDGRAVVFSVDYRLAPEHKFPAAVEDAYDALQWIAERAADFHLDPARIAVGGDSAGGNLAAVTSILAKERGGPAIAFQLLIYPFTGYDPAHPPASILENAEGYLLTGGMMLWFRDQYLNSLEELTHPWFSPVLYPDLSGLPPAYIATAQYDPLRDVGKLYAEALNKAGVKVEIENFEDLIHGFASFYSLSPGATKALVRIAEKLRDALA

SEQ ID NO: 57 - DNA, 930 bp, synthetic construct
  misc_feature 1..930: note = Description of Artificial Sequence: Syntheticpolynucleotide sequence encoding a codon optimizedcarboxyesterase enzyme
  source 1..930: mol_type = other DNA
atgccattagatcctgtgattcaatatgtcctcgatcaactgaaccgtatgccagcccctgactacaagcacttaagcgctcaacaggttcgttcacagcaacacctgtttccaccagttaagaaagaaccggtcgcagaagttcgcgaattcgacatggatctgccgggccgtaccctgaaagtccgtatgtaccgcccggaaggtgttgaaccaccatatccagcactggtttactaccatggtggcggttgggttgcgggtgacctggaaacgcatgatccggtgtgtcgtgtgttggcgaaagatggacgcgcagtggtgtttagcgttgactaccgtctggcaccagaacacaagtttccagcggcagttgaagacgcgtatgatgcactgcaatggattgcagaacgtgcagccgatttccatcttgatccagcacgcattgcagttggcggcgattcagcaggcggcaacctggcggccgtgactagtattctggcgaaagaacgtggtggtccagcaattgcgtttcaactgctgatctatccctttactggttatgatccagcacatccaccagcaagtatccttgagaatgcggagggttacctgttaaccggaggcatgatgctgtggtttcgtgaccagtacctgaacagccttgaggaactgactcacccatggtttagtccagtgctgtacccggatcttagcggtttaccaccggcgtacattgcaaccgcacagtacgatcccctgcgcgatgtcggcaaactttacgctgaagccctgaacaaagcgggcgttaaggtggagatcgagaacttcgaggatctgattcatggcttcgcgcagttctattctctgagcccaggcgcaaccaaagcactggtacgtattgccgagaaactgcgcgatgcgttggcg

SEQ ID NO: 58 - protein, 310 aa, synthetic construct
  REGION 1..310: note = Description of Artificial Sequence: Syntheticpolypeptide sequence of a codon optimizedcarboxyesterase enzyme
MPLDPVIQYVLDQLNRMPAPDYKHLSAQQVRSQQHLFPPVKKEPVAEVREFDMDLPGRTLKVRMYRPEGVEPPYPALVYYHGGGWVAGDLETHDPVCRVLAKDGRAVVFSVDYRLAPEHKFPAAVEDAYDALQWIAERAADFHLDPARIAVGGDSAGGNLAAVTSILAKERGGPAIAFQLLIYPFTGYDPAHPPASILENAEGYLLTGGMMLWFRDQYLNSLEELTHPWFSPVLYPDLSGLPPAYIATAQYDPLRDVGKLYAEALNKAGVKVEIENFEDLIHGFAQFYSLSPGATKALVRIAEKLRDALA

SEQ ID NO: 59 - DNA, 930 bp, synthetic construct
  misc_feature 1..930: note = Description of Artificial Sequence: Syntheticpolynucleotide sequence encoding a codon optimizedcarboxyesterase enzyme
  source 1..930: mol_type = other DNA
atgccattagatcctgtgattcaatatgtcctcgatcaactgaaccgtatgccagcccctgactacaagcacttaagcgctcaacagtttcgttcacaggaacacctgtttccaccagttaagaaagaaccggtcgcagaagttcgcgaattcgacatggatctgccgggccgtaccctgaaagtccgtatgtaccgcccggaaggtgttgaaccaccatatccagcactggtttactaccatggtggcggttgggttgcgggtgacctggaaacgcatgatccggtgtgtcgtgtgttggcgaaagatggacgcgcagtggtgtttagcgttgactaccgtctggcaccagaacacaagtttccagcggcagttgaagacgcgtatgatgcactgcaatggattgcagaacgtgcagccgatttccatcttgatccagcacgcattgcagttggcggcgattcagcaggcggcaacctggcggccgtgactagtattctggcgaaagaacgtggtggtccagcaattgcgtttcaactgctgatctatccctttactggttatgatccagcacatccaccagcaagtatccttgagaatgcggagggttacctgttaaccggaggcatgatgctgtggtttcgtgaccagtacctgaacagccttgaggaactgactcacccatggtttagtccagtgctgtacccggatcttagcggtttaccaccggcgtacattgcaaccgcacagtacgatcccctgcgcgatgtcggcaaactttacgctgaagccctgaacaaagcgggcgttaaggtggagatcgagaacttcgaggatctgattcatggcttcgcgcagttctattctctgagcccaggcgcaaccaaagcactggtacgtattgccgagaaactgcgcgatgcgttggcg

SEQ ID NO: 60 - protein, 310 aa, synthetic construct
  REGION 1..310: note = Description of Artificial Sequence: Syntheticpolypeptide sequence of a codon optimizedcarboxyesterase enzyme
MPLDPVIQYVLDQLNRMPAPDYKHLSAQQFRSQEHLFPPVKKEPVAEVREFDMDLPGRTLKVRMYRPEGVEPPYPALVYYHGGGWVAGDLETHDPVCRVLAKDGRAVVFSVDYRLAPEHKFPAAVEDAYDALQWIAERAADFHLDPARIAVGGDSAGGNLAAVTSILAKERGGPAIAFQLLIYPFTGYDPAHPPASILENAEGYLLTGGMMLWFRDQYLNSLEELTHPWFSPVLYPDLSGLPPAYIATAQYDPLRDVGKLYAEALNKAGVKVEIENFEDLIHGFAQFYSLSPGATKALVRIAEKLRDALA

SEQ ID NO: 61 - DNA, 930 bp, synthetic construct
  misc_feature 1..930: note = Description of Artificial Sequence: Syntheticpolynucleotide sequence encoding a codon optimizedcarboxyesterase enzyme
  source 1..930: mol_type = other DNA
atgccattagatcctgtgattcaatatgtcctcgatcaactgaaccgtatgccagcccctgactacaagcacttaagcgctcaacagtttcgttcacagcaacacctgtttccaccagttaagaaagaaccggtcgcagaagttcgcgaattcgacatggatctgccgggccgtaccctgaaagtccgtatgtaccgcccggaaggtgttgaaccaccatatccagcactggtttactaccatggtggcggttgggttgcgggtgacctggaaacgcatgatccggtgtgtcgtgtgttggcgaaagatggacgcgcagtggtgtttagcgttgactaccgtctggcaccagaacacaagtttccagcggcagttgaagacgcgtatgatgcactgcaatggattgcagaacgtgcagccgatttccatcttgatccagcacgcattgcagttggcggcgattcagcaggcggcaacctggcggccgtgactagtattctggcgaaagaacgtggtggtccagcaattgcgtttcaactgctgatctatccctttactggttttgatccagcacatccaccagcaagtatccttgagaatgcggagggttacctgttaaccggaggcatgatgctgtggtttcgtgaccagtacctgaacagccttgaggaactgactcacccatggtttagtccagtgctgtacccggatcttagcggtttaccaccggcgtacattgcaaccgcacagtacgatcccctgcgcgatgtcggcaaactttacgctgaagccctgaacaaagcgggcgttaaggtggagatcgagaacttcgaggatctgattcatggcttcgcgcagttctattctctgagcccaggcgcaaccaaagcactggtacgtattgccgagaaactgcgcgatgcgttggcg

SEQ ID NO: 62 - protein, 310 aa, synthetic construct
  REGION 1..310: note = Description of Artificial Sequence: Syntheticpolypeptide sequence of a codon optimizedcarboxyesterase enzyme
MPLDPVIQYVLDQLNRMPAPDYKHLSAQQFRSQQHLFPPVKKEPVAEVREFDMDLPGRTLKVRMYRPEGVEPPYPALVYYHGGGWVAGDLETHDPVCRVLAKDGRAVVFSVDYRLAPEHKFPAAVEDAYDALQWIAERAADFHLDPARIAVGGDSAGGNLAAVTSILAKERGGPAIAFQLLIYPFTGFDPAHPPASILENAEGYLLTGGMMLWFRDQYLNSLEELTHPWFSPVLYPDLSGLPPAYIATAQYDPLRDVGKLYAEALNKAGVKVEIENFEDLIHGFAQFYSLSPGATKALVRIAEKLRDALA

SEQ ID NO: 63 - DNA, 930 bp, synthetic construct
  misc_feature 1..930: note = Description of Artificial Sequence: Syntheticpolynucleotide sequence encoding a codon optimizedcarboxyesterase enzyme
  source 1..930: mol_type = other DNA
atgccattagatcctgtgattcaatatgtcctcgatcaactgaaccgtatgccagcccctgactacaagcacttaagcgctcaacagtttcgttcacagcaacacctgtttccaccagttaagaaagaaccggtcgcagaagttcgcgaattcgacatggatctgccgggccgtaccctgaaagtccgtatgtaccgcccggaaggtgttgaaccaccatatccagcactggtttactaccatggtggcggttgggttgcgggtgacctggaaacgcatgatccggtgtgtcgtgtgttggcgaaagatggacgcgcagtggtgtttagcgttgactaccgtctggcaccagaacacaagtttccagcggcagttgaagacgcgtatgatgcactgcaatggattgcagaacgtgcagccgatttccatcttgatccagcacgcattgcagttggcggcgattcagcaggcggcaacctggcggccgtgactagtattctggcgaaagaacgtggtggtccagcaattgcgtttcaactgctgatctatccctttactggttatgatccagcacatccaccagcaagtatccttgagaatgcggagggttacctgttaaccggaggcatgatgctgtggtttcgtattcagtacctgaacagccttgaggaactgactcacccatggtttagtccagtgctgtacccggatcttagcggtttaccaccggcgtacattgcaaccgcacagtacgatcccctgcgcgatgtcggcaaactttacgctgaagccctgaacaaagcgggcgttaaggtggagatcgagaacttcgaggatctgattcatggcttcgcgcagttctattctctgagcccaggcgcaaccaaagcactggtacgtattgccgagaaactgcgcgatgcgttggcg

SEQ ID NO: 64 - protein, 310 aa, synthetic construct
  REGION 1..310: note = Description of Artificial Sequence: Syntheticpolypeptide sequence of a codon optimizedcarboxyesterase enzyme
MPLDPVIQYVLDQLNRMPAPDYKHLSAQQFRSQQHLFPPVKKEPVAEVREFDMDLPGRTLKVRMYRPEGVEPPYPALVYYHGGGWVAGDLETHDPVCRVLAKDGRAVVFSVDYRLAPEHKFPAAVEDAYDALQWIAERAADFHLDPARIAVGGDSAGGNLAAVTSILAKERGGPAIAFQLLIYPFTGYDPAHPPASILENAEGYLLTGGMMLWFRIQYLNSLEELTHPWFSPVLYPDLSGLPPAYIATAQYDPLRDVGKLYAEALNKAGVKVEIENFEDLIHGFAQFYSLSPGATKALVRIAEKLRDALA

SEQ ID NO: 65 - DNA, 930 bp, synthetic construct
  misc_feature 1..930: note = Description of Artificial Sequence: Syntheticpolynucleotide sequence encoding a codon optimizedcarboxyesterase enzyme
  source 1..930: mol_type = other DNA
atgccattagatcctgtgattcaatatgtcctcgatcaactgaaccgtatgccagccattgactacaagcacttaagcgctcaacagtttcgttcacagcaacacctgtttccaccagttaagaaagaaccggtcgcagaagttcgcgaattcgacatggatctgccgggccgtaccctgaaagtccgtatgtaccgcccggaaggtgttgaaccaccatatccagcactggtttactaccatggtggcggttgggttgcgggtgacctggaaacgcatgatccggtgtgtcgtgtgttggcgaaagatggacgcgcagtggtgtttagcgttgactaccgtctggcaccagaacacaagtttccagcggcagttgaagacgcgtatgatgcactgcaatggattgcagaacgtgcagccgatttccatcttgatccagcacgcattgcagttggcggcgattcagcaggcggcaacctggcggccgtgactagtattctggcgaaagaacgtggtggtccagcaattgcgtttcaactgctgatctatccctttactggttatgatccagcacatccaccagcaagtatccttgagaatgcggagggttacctgttaaccggaggcatgatgctgtggtttcgtgaccagtacctgaacagccttgaggaactgactcacccatggtttagtccagtgctgtacccggatcttagcggtttaccaccggcgtacattgcaaccgcacagtacgatcccctgcgcgatgtcggcaaactttacgctgaagccctgaacaaagcgggcgttaaggtggagatcgagaacttcgaggatctgattcatggcttcgcgcagttctattctctgagcccaggcgcaaccaaagcactggtacgtattgccgagaaactgcgcgatgcgttggcg

SEQ ID NO: 66 - protein, 310 aa, synthetic construct
  REGION 1..310: note = Description of Artificial Sequence: Syntheticpolypeptide sequence of a codon optimizedcarboxyesterase enzyme
MPLDPVIQYVLDQLNRMPAIDYKHLSAQQFRSQQHLFPPVKKEPVAEVREFDMDLPGRTLKVRMYRPEGVEPPYPALVYYHGGGWVAGDLETHDPVCRVLAKDGRAVVFSVDYRLAPEHKFPAAVEDAYDALQWIAERAADFHLDPARIAVGGDSAGGNLAAVTSILAKERGGPAIAFQLLIYPFTGYDPAHPPASILENAEGYLLTGGMMLWFRDQYLNSLEELTHPWFSPVLYPDLSGLPPAYIATAQYDPLRDVGKLYAEALNKAGVKVEIENFEDLIHGFAQFYSLSPGATKALVRIAEKLRDALA

SEQ ID NO: 67 - DNA, 930 bp, synthetic construct
  misc_feature 1..930: note = Description of Artificial Sequence: Syntheticpolynucleotide sequence encoding a codon optimizedcarboxyesterase enzyme
  source 1..930: mol_type = other DNA
atgccattagatcctgtgattcaatatgtcctcgatcaactgaaccgtatgccagcccctgactacaagcacttaagcgctcaacagtttcgttcacagcaacacctgtttccaccagttaagaaagaaccggtcgcagaagttcgcgaattcgacatggatctgccgggccgtaccctgaaagtccgtatgtaccgcccggaaggtgttgaaccaccatatccagcactggtttactaccatggtggcggttgggttgcgggtgacctggaaacgcatgatccggtgtgtcgtgtgttggcgaaagatggacgcgcagtggtgtttagcgttgactaccgtctggcaccagaacacaagtttccagcggcagttgaagacgcgtatgatgcactgcaatggattgcagaacgtgcagccgatttccatcttgatccagcacgcattgcagttggcggcgattcagcaggcggcaacctggcggccgtgactagtattctggcgaaagaacgtggtggtccagcaattgcgtttcaactgctgatctatccctttactggttatgatccagcacatccaccagcaagtatccttgagaatgcggagggttacctgttaaccggaggcatgatgctgtggtttcgtaatcagtacctgaacagccttgaggaactgactcacccatggtttagtccagtgctgtacccggatcttagcggtttaccaccggcgtacattgcaaccgcacagtacgatcccctgcgcgatgtcggcaaactttacgctgaagccctgaacaaagcgggcgttaaggtggagatcgagaacttcgaggatctgattcatggcttcgcgcagttctattctctgagcccaggcgcaaccaaagcactggtacgtattgccgagaaactgcgcgatgcgttggcg

SEQ ID NO: 68 - protein, 310 aa, synthetic construct
  REGION 1..310: note = Description of Artificial Sequence: Syntheticpolypeptide sequence of a codon optimizedcarboxyesterase enzyme
MPLDPVIQYVLDQLNRMPAPDYKHLSAQQFRSQQHLFPPVKKEPVAEVREFDMDLPGRTLKVRMYRPEGVEPPYPALVYYHGGGWVAGDLETHDPVCRVLAKDGRAVVFSVDYRLAPEHKFPAAVEDAYDALQWIAERAADFHLDPARIAVGGDSAGGNLAAVTSILAKERGGPAIAFQLLIYPFTGYDPAHPPASILENAEGYLLTGGMMLWFRNQYLNSLEELTHPWFSPVLYPDLSGLPPAYIATAQYDPLRDVGKLYAEALNKAGVKVEIENFEDLIHGFAQFYSLSPGATKALVRIAEKLRDALA

SEQ ID NO: 69 - DNA, 930 bp, synthetic construct
  misc_feature 1..930: note = Description of Artificial Sequence: Syntheticpolynucleotide sequence encoding a codon optimizedcarboxyesterase enzyme
  source 1..930: mol_type = other DNA
atgccattagatcctgtgattcaatatgtcctcgatcaactgaaccgtatgccagcccctgactacaagcacttaagcgctcaagattttcgttcacagcaacacctgtttccaccagttaagaaagaaccggtcgcagaagttcgcgaattcgacatggatctgccgggccgtaccctgaaagtccgtatgtaccgcccggaaggtgttgaaccaccatatccagcactggtttactaccatggtggcggttgggttgcgggtgacctggaaacgcatgatccggtgtgtcgtgtgttggcgaaagatggacgcgcagtggtgtttagcgttgactaccgtctggcaccagaacacaagtttccagcggcagttgaagacgcgtatgatgcactgcaatggattgcagaacgtgcagccgatttccatcttgatccagcacgcattgcagttggcggcgattcagcaggcggcaacctggcggccgtgactagtattctggcgaaagaacgtggtggtccagcaattgcgtttcaactgctgatctatccctttactggttatgatccagcacatccaccagcaagtatccttgagaatgcggagggttacctgttaaccggaggcatgatgctgtggtttcgtgaccagtacctgaacagccttgaggaactgactcacccatggtttagtccagtgctgtacccggatcttagcggtttaccaccggcgtacattgcaaccgcacagtacgatcccctgcgcgatgtcggcaaactttacgctgaagccctgaacaaagcgggcgttaaggtggagatcgagaacttcgaggatctgattcatggcttcgcgcagttctattctctgagcccaggcgcaaccaaagcactggtacgtattgccgagaaactgcgcgatgcgttggcg

SEQ ID NO: 70 - protein, 310 aa, synthetic construct
  REGION 1..310: note = Description of Artificial Sequence: Syntheticpolypeptide sequence of a codon optimizedcarboxyesterase enzyme
MPLDPVIQYVLDQLNRMPAPDYKHLSAQDFRSQQHLFPPVKKEPVAEVREFDMDLPGRTLKVRMYRPEGVEPPYPALVYYHGGGWVAGDLETHDPVCRVLAKDGRAVVFSVDYRLAPEHKFPAAVEDAYDALQWIAERAADFHLDPARIAVGGDSAGGNLAAVTSILAKERGGPAIAFQLLIYPFTGYDPAHPPASILENAEGYLLTGGMMLWFRDQYLNSLEELTHPWFSPVLYPDLSGLPPAYIATAQYDPLRDVGKLYAEALNKAGVKVEIENFEDLIHGFAQFYSLSPGATKALVRIAEKLRDALA

SEQ ID NO: 71 - DNA, 930 bp, synthetic construct
  misc_feature 1..930: note = Description of Artificial Sequence: Syntheticpolynucleotide sequence encoding a codon optimizedcarboxyesterase enzyme
  source 1..930: mol_type = other DNA
atgccattagatcctgtgattcaatatgtcctcgatcaactgaaccgtatgccagcccctgactacaagcacttaagcgctcaacagtttcgttcaggtcaacacctgtttccaccagttaagaaagaaccggtcgcagaagttcgcgaattcgacatggatctgccgggccgtaccctgaaagtccgtatgtaccgcccggaaggtgttgaaccaccatatccagcactggtttactaccatggtggcggttgggttgcgggtgacctggaaacgcatgatccggtgtgtcgtgtgttggcgaaagatggacgcgcagtggtgtttagcgttgactaccgtctggcaccagaacacaagtttccagcggcagttgaagacgcgtatgatgcactgcaatggattgcagaacgtgcagccgatttccatcttgatccagcacgcattgcagttggcggcgattcagcaggcggcaacctggcggccgtgactagtattctggcgaaagaacgtggtggtccagcaattgcgtttcaactgctgatctatccctttactggttatgatccagcacatccaccagcaagtatccttgagaatgcggagggttacctgttaaccggaggcatgatgctgtggtttcgtgaccagtacctgaacagccttgaggaactgactcacccatggtttagtccagtgctgtacccggatcttagcggtttaccaccggcgtacattgcaaccgcacagtacgatcccctgcgcgatgtcggcaaactttacgctgaagccctgaacaaagcgggcgttaaggtggagatcgagaacttcgaggatctgattcatggcttcgcgcagttctattctctgagcccaggcgcaaccaaagcactggtacgtattgccgagaaactgcgcgatgcgttggcg

SEQ ID NO: 72 - protein, 310 aa, synthetic construct
  REGION 1..310: note = Description of Artificial Sequence: Syntheticpolypeptide sequence of a codon optimizedcarboxyesterase enzyme
MPLDPVIQYVLDQLNRMPAPDYKHLSAQQFRSGQHLFPPVKKEPVAEVREFDMDLPGRTLKVRMYRPEGVEPPYPALVYYHGGGWVAGDLETHDPVCRVLAKDGRAVVFSVDYRLAPEHKFPAAVEDAYDALQWIAERAADFHLDPARIAVGGDSAGGNLAAVTSILAKERGGPAIAFQLLIYPFTGYDPAHPPASILENAEGYLLTGGMMLWFRDQYLNSLEELTHPWFSPVLYPDLSGLPPAYIATAQYDPLRDVGKLYAEALNKAGVKVEIENFEDLIHGFAQFYSLSPGATKALVRIAEKLRDALA

SEQ ID NO: 73 - DNA, 930 bp, synthetic construct
  misc_feature 1..930: note = Description of Artificial Sequence: Syntheticpolynucleotide sequence encoding a codon optimizedcarboxyesterase enzyme
  source 1..930: mol_type = other DNA
atgccattagatcctgtgattcaatatgtcctcgatcaactgaaccgtatgccagcccctgactacaagcacttaagcgctagtcagtttcgttcacagcaacacctgtttccaccagttaagaaagaaccggtcgcagaagttcgcgaattcgacatggatctgccgggccgtaccctgaaagtccgtatgtaccgcccggaaggtgttgaaccaccatatccagcactggtttactaccatggtggcggttgggttgcgggtgacctggaaacgcatgatccggtgtgtcgtgtgttggcgaaagatggacgcgcagtggtgtttagcgttgactaccgtctggcaccagaacacaagtttccagcggcagttgaagacgcgtatgatgcactgcaatggattgcagaacgtgcagccgatttccatcttgatccagcacgcattgcagttggcggcgattcagcaggcggcaacctggcggccgtgactagtattctggcgaaagaacgtggtggtccagcaattgcgtttcaactgctgatctatccctttactggttatgatccagcacatccaccagcaagtatccttgagaatgcggagggttacctgttaaccggaggcatgatgctgtggtttcgtgaccagtacctgaacagccttgaggaactgactcacccatggtttagtccagtgctgtacccggatcttagcggtttaccaccggcgtacattgcaaccgcacagtacgatcccctgcgcgatgtcggcaaactttacgctgaagccctgaacaaagcgggcgttaaggtggagatcgagaacttcgaggatctgattcatggcttcgcgcagttctattctctgagcccaggcgcaaccaaagcactggtacgtattgccgagaaactgcgcgatgcgttggcg

SEQ ID NO: 74 - protein, 310 aa, synthetic construct
  REGION 1..310: note = Description of Artificial Sequence: Syntheticpolypeptide sequence of a codon optimizedcarboxyesterase enzyme
MPLDPVIQYVLDQLNRMPAPDYKHLSASQFRSQQHLFPPVKKEPVAEVREFDMDLPGRTLKVRMYRPEGVEPPYPALVYYHGGGWVAGDLETHDPVCRVLAKDGRAVVFSVDYRLAPEHKFPAAVEDAYDALQWIAERAADFHLDPARIAVGGDSAGGNLAAVTSILAKERGGPAIAFQLLIYPFTGYDPAHPPASILENAEGYLLTGGMMLWFRDQYLNSLEELTHPWFSPVLYPDLSGLPPAYIATAQYDPLRDVGKLYAEALNKAGVKVEIENFEDLIHGFAQFYSLSPGATKALVRIAEKLRDALA

SEQ ID NO: 75 - DNA, 930 bp, synthetic construct
  misc_feature 1..930: note = Description of Artificial Sequence: Syntheticpolynucleotide sequence encoding a codon optimizedcarboxyesterase enzyme
  source 1..930: mol_type = other DNA
atgccattagatcctgtgattcaatatgtgctcgatcaactgaaccgtatgccagcccctgactacaagcacttaagcgctcaacaggttcgttcacaacaacacctgtttccaccagttaagaaagaaccggtcgcagaagttcgcgaattcgacatggatctgccgggccgtaccctgaaagtccgtatgtaccgcccggaaggtgttgaaccaccatatccagcactggtttactaccatggtggcggttgggttgcgggtgacctggaaacgcatgatccggtgtgtcgtgtgttggcgaaagatggacgcgcagtggtgtttagcgttgactaccgtctggcaccagaacacaagtttccagcggcagttgaagacgcgtatgatgcactgcaatggattgcagaacgtgcagccgatttccatcttgatccagcacgcattgcagttggcggcgattcagcaggcggcaacctggcggccgtgactagtattctggcgaaagaacgtggtggtccagcaattgcgtttcaactgctgatctatccctttactggttatgatccagcacatccaccagcaagtcttcttgagaatgcggagggttacctgttaaccggaggcatgatgctgtggtttcgtaatcagtacctgaacagccttgaggaactgactcacccatggtttagtccagtgctgtacccggatcttagcggtttaccaccggcgtacattgcaaccgcacagtacgatcccctgcgcgatgtcggcaaactttacgctgaagccctgaacaaagcgggcgttaaggtggagatcgagaacttcgaggatctgattcatggcttcgcgcagttctattctctgagcccaggcgcaaccaaagcactggtacgtattgccgagaaactgcgcgatgcgttggcg

SEQ ID NO: 76 - protein, 310 aa, synthetic construct
  REGION 1..310: note = Description of Artificial Sequence: Syntheticpolypeptide sequence of a codon optimizedcarboxyesterase enzyme
MPLDPVIQYVLDQLNRMPAPDYKHLSAQQVRSQQHLFPPVKKEPVAEVREFDMDLPGRTLKVRMYRPEGVEPPYPALVYYHGGGWVAGDLETHDPVCRVLAKDGRAVVFSVDYRLAPEHKFPAAVEDAYDALQWIAERAADFHLDPARIAVGGDSAGGNLAAVTSILAKERGGPAIAFQLLIYPFTGYDPAHPPASLLENAEGYLLTGGMMLWFRNQYLNSLEELTHPWFSPVLYPDLSGLPPAYIATAQYDPLRDVGKLYAEALNKAGVKVEIENFEDLIHGFAQFYSLSPGATKALVRIAEKLRDALA

SEQ ID NO: 77 - DNA, 930 bp, synthetic construct
  misc_feature 1..930: note = Description of Artificial Sequence: Syntheticpolynucleotide sequence encoding a codon optimizedcarboxyesterase enzyme
  source 1..930: mol_type = other DNA
atgccattagatcctgtgattcaatatgtgctcgatcaactgaaccgtatgccagcccctgactacaagcacttaagcgctcaacagtttcgttcacagcaacacattggtccaccagttaagaaagaaccggtcgcagaagttcgcgaattcgacatggatctgccgggccgtaccctgaaagtccgtatgtaccgcccggaaggtgttgaaccaccatatccagcactggtttactaccatggtggcggttgggttgcgggtgacctggaaacgcatgatccggtgtgtcgtgtgttggcgaaagatggacgcgcagtggtgtttagcgttgactaccgtctggcaccagaacacaagtttccagcggcagttgaagacgcgtatgatgcactgcaatggattgcagaacgtgcagccgatttccatcttgatccagcacgcattgcagttggcggcgattcagcaggcggcaacctggcggccgtgactagtattctggcgaaagaacgtggtggtccagcaattgcgtttcaactgctgatctatccctttactggttatgatccagcacatccaccagcaagtatccttgagaatgcggagggttacctgttaaccggaggcatgatgctgtggtttcgtaatcagtacctgaacagccttgaggaactgactcacccatggtttagtccagtgctgtacccggatcttagcggtttaccaccggcgtacattgcaaccgcacagtacgatcccctgcgcgatgtcggcaaactttacgctgaagccctgaacaaagcgggcgttaaggtggagatcgagaacttcgaggatacgattcatggcttcgcgcagttttattctattagcccaggcgcaaccaaagcactggtacgtattgccgagaaactgcgcgatgcgttggcg

SEQ ID NO: 78 - protein, 310 aa, synthetic construct
  REGION 1..310: note = Description of Artificial Sequence: Syntheticpolypeptide sequence of a codon optimizedcarboxyesterase enzyme
MPLDPVIQYVLDQLNRMPAPDYKHLSAQQFRSQQHIGPPVKKEPVAEVREFDMDLPGRTLKVRMYRPEGVEPPYPALVYYHGGGWVAGDLETHDPVCRVLAKDGRAVVFSVDYRLAPEHKFPAAVEDAYDALQWIAERAADFHLDPARIAVGGDSAGGNLAAVTSILAKERGGPAIAFQLLIYPFTGYDPAHPPASILENAEGYLLTGGMMLWFRNQYLNSLEELTHPWFSPVLYPDLSGLPPAYIATAQYDPLRDVGKLYAEALNKAGVKVEIENFEDTIHGFAQFYSISPGATKALVRIAEKLRDALA

SEQ ID NO: 79 - DNA, 930 bp, synthetic construct
  misc_feature 1..930: note = Description of Artificial Sequence: Syntheticpolynucleotide sequence encoding a codon optimizedcarboxyesterase enzyme
  source 1..930: mol_type = other DNA
atgccattagatcctgtgattcaatatgtcctcgatcaactgaaccgtatgccagcccctgactacaagcacttaagcgctcaacagtttcgttcacagcaacacatgggtccaccagttaagaaagaaccggtcgcagaagttcgcgaattcgacatggatctgccgggccgtaccctgaaagtccgtatgtaccgcccggaaggtgttgaaccaccatatccagcactggtttactaccatggtggcggttgggttgcgggtgacctggaaacgcatgatccggtgtgtcgtgtgttggcgaaagatggacgcgcagtggtgtttagcgttgactaccgtctggcaccagaacacaagtttccagcggcagttgaagacgcgtatgatgcactgcaatggattgcagaacgtgcagccgatttccatcttgatccagcacgcattgcagttggcggcgattcagcaggcggcaacctggcggccgtgactagtattctggcgaaagaacgtggtggtccagcaattgcgtttcaactgctgatctatccctttactggttatgatccagcacatccaccagcaagtatccttgagaatgcggagggttacctgttaaccggaggcatgatgctgtggtttcgtaatcagtacctgaacagccttgaggaactgactcacccatggtttagtccagtgctgtacccggatcttagcggtttaccaccggcgtacattgcaaccgcacagtacgatcccctgcgcgatgtcggcaaactttacgctgaagccctgaacaaagcgggcgttaaggtggagatcgagaacttcgaggatatgattcatggcttcgcgcagttctattctattagcccaggcgcaaccaaagcactggtacgtattgccgagaaactgcgcgatgcgttggcg

SEQ ID NO: 80 - protein, 310 aa, synthetic construct
  REGION 1..310: note = Description of Artificial Sequence: Syntheticpolypeptide sequence of a codon optimizedcarboxyesterase enzyme
MPLDPVIQYVLDQLNRMPAPDYKHLSAQQFRSQQHMGPPVKKEPVAEVREFDMDLPGRTLKVRMYRPEGVEPPYPALVYYHGGGWVAGDLETHDPVCRVLAKDGRAVVFSVDYRLAPEHKFPAAVEDAYDALQWIAERAADFHLDPARIAVGGDSAGGNLAAVTSILAKERGGPAIAFQLLIYPFTGYDPAHPPASILENAEGYLLTGGMMLWFRNQYLNSLEELTHPWFSPVLYPDLSGLPPAYIATAQYDPLRDVGKLYAEALNKAGVKVEIENFEDMIHGFAQFYSISPGATKALVRIAEKLRDALA

SEQ ID NO: 81 - DNA, 930 bp, synthetic construct
  misc_feature 1..930: note = Description of Artificial Sequence: Syntheticpolynucleotide sequence encoding a codon optimizedcarboxyesterase enzyme
  source 1..930: mol_type = other DNA
atgccattagatcctgtgattcaatatatgctcgatcaactgaaccgtatgccagcccctgactacaagcacttaagcgctcaacagtttcgttcacagcaacacttgggtccaccagttaagaaagaaccggtcgcagaagttcgcgaattcgacatggatctgccgggccgtaccctgaaagtccgtatgtaccgcccggaaggtgttgaaccaccatatccagcactggtttactaccatggtggcggttgggttgcgggtgacctggaaacgcatgatccggtgtgtcgtgtgttggcgaaagatggacgcgcagtggtgtttagcgttgactaccgtctggcaccagaacacaagtttccagcggcagttgaagacgcgtatgatgcactgcaatggattgcagaacgtgcagccgatttccatcttgatccagcacgcattgcagttggcggcgattcagcaggcggcaacctggcggccgtgactagtattctggcgaaagaacgtggtggtccagcaattgcgtttcaactgctgatctatccctttactggttatgatccagcacatccaccagcaagtatccttgagaatgcggagggttacctgttaaccggaggcatgatgctgtggtttcgtaatcagtacctgaacagccttgaggaactgactcacccatggtttagtccagtgctgtacccggatcttagcggtttaccaccggcgtacattgcaaccgcacagtacgatcccctgcgcgatgtcggcaaactttacgctgaagccctgaacaaagcgggcgttaaggtggagatcgagaacttcgaggatctaattcatggcttcgcgcagttctattctctgagcccaggcgcaaccaaagcactggtacgtattgccgagaaactgcgcgatgcgttggcg

SEQ ID NO: 82 - protein, 310 aa, synthetic construct
  REGION 1..310: note = Description of Artificial Sequence: Syntheticpolypeptide sequence of a codon optimizedcarboxyesterase enzyme
MPLDPVIQYMLDQLNRMPAPDYKHLSAQQFRSQQHLGPPVKKEPVAEVREFDMDLPGRTLKVRMYRPEGVEPPYPALVYYHGGGWVAGDLETHDPVCRVLAKDGRAVVFSVDYRLAPEHKFPAAVEDAYDALQWIAERAADFHLDPARIAVGGDSAGGNLAAVTSILAKERGGPAIAFQLLIYPFTGYDPAHPPASILENAEGYLLTGGMMLWFRNQYLNSLEELTHPWFSPVLYPDLSGLPPAYIATAQYDPLRDVGKLYAEALNKAGVKVEIENFEDLIHGFAQFYSLSPGATKALVRIAEKLRDALA

SEQ ID NO: 83 - DNA, 930 bp, synthetic construct
  misc_feature 1..930: note = Description of Artificial Sequence: Syntheticpolynucleotide sequence encoding a codon optimizedcarboxyesterase enzyme
  source 1..930: mol_type = other DNA
atgccattagatcctgtgattcaatatgtcctcgatcaactgaaccgtatgccagcccctgactacaagcacttaagcgctagtcagtttcgttcacagcaacacctgtttccaccagttaagaaagaaccggtcgcagaagttcgcgaattcgacatggatctgccgggccgtaccctgaaagtccgtatgtaccgcccggaaggtgttgaaccaccatatccagcactggtttactaccatggtggcggttgggttgcgggtgacctggaaacgcatgatccggtgtgtcgtgtgttggcgaaagatggacgcgcagtggtgtttagcgttgactaccgtctggcaccagaacacaagtttccagcggcagttgaagacgcgtatgatgcactgcaatggattgcagaacgtgcagccgatttccatcttgatccagcacgcattgcagttggcggcgattcagcaggcggcaacctggcggccgtgactagtattctggcgaaagaacgtggtggtccagcaattgcgtttcaactgctgatctatccctttactggttacgatccagcacatccaccagcaagtattcttgagaatgcggagggttacctgttaaccggaggcatgatgctgtggtttcgtaatcagtacctgaacagccttgaggaactgactcacccatggtttagtccagtgctgtacccggatcttagcggtttaccaccggcgtacattgcaaccgcacagtacgatcccctgcgcgatgtcggtaaactttacgctgaagccctgaacaaagcgggcgttaaggtggagatcgagaacttcgaggatctgattcatggcttcgcgcagttctattctctgagcccaggcgcaaccaaagcactggtacgtattgccgagaaactgcgcgatgcgttggcg

SEQ ID NO: 84 - protein, 310 aa, synthetic construct
  REGION 1..310: note = Description of Artificial Sequence: Syntheticpolypeptide sequence of a codon optimizedcarboxyesterase enzyme
MPLDPVIQYVLDQLNRMPAPDYKHLSASQFRSQQHLFPPVKKEPVAEVREFDMDLPGRTLKVRMYRPEGVEPPYPALVYYHGGGWVAGDLETHDPVCRVLAKDGRAVVFSVDYRLAPEHKFPAAVEDAYDALQWIAERAADFHLDPARIAVGGDSAGGNLAAVTSILAKERGGPAIAFQLLIYPFTGYDPAHPPASILENAEGYLLTGGMMLWFRNQYLNSLEELTHPWFSPVLYPDLSGLPPAYIATAQYDPLRDVGKLYAEALNKAGVKVEIENFEDLIHGFAQFYSLSPGATKALVRIAEKLRDALA

SEQ ID NO: 85 - DNA, 930 bp, synthetic construct
  misc_feature 1..930: note = Description of Artificial Sequence: Syntheticpolynucleotide sequence encoding a codon optimizedcarboxyesterase enzyme
  source 1..930: mol_type = other DNA
atgccattagatcctgtgattcaatatgtcctcgatcaactgaaccgtatgccagcccctgactacaagcacttaagcgctagtcagtttcgttcacagcaacatctgtttccaccagttaagaaagaaccggtcgcagaagttcgcgaattcgacatggatctgccgggccgtaccctgaaagtccgtatgtaccgcccggaaggtgttgaaccaccatatccagcactggtttactaccatggtggcggttgggttgcgggtgacctggaaacgcatgatccggtgtgtcgtgtgttggcgaaagatggacgcgcagtggtgtttagcgttgactaccgtctggcaccagaacacaagtttccagcggcagttgaagacgcgtatgatgcactgcaatggattgcagaacgtgcagccgatttccatcttgatccagcacgcattgcagttggcggcgattcagcgggcggcaacctggcggccgtgactagtattctggcgaaagaacgtggtggtccagcaattgcgtttcaactgctgatctatccctttactggttacgatccagcacatccaccagcaagtcttcttgagaatgcggagggttacctgttaaccggaggcatgatgctgtggtttcgtaatcagtacctgaacagccttgaggaactgactcacccatggtttagtccagtgctgtacccggatcttagcggtttaccaccggcgtacattgcaaccgcacagtacgatcccctgcgcgatgtcggtaaactttacgctgaagccctgaccaaagcgggcgttaaggtggagatcgagaacttcgaggatctgattcatggcttcgcgcagttctattctctgagcccaggcgcaaccaaagcactggtacgtattgccgagaaactgcgcgatgcgttggcg

SEQ ID NO: 86 - protein, 310 aa, synthetic construct
  REGION 1..310: note = Description of Artificial Sequence: Syntheticpolypeptide sequence of a codon optimizedcarboxyesterase enzyme
MPLDPVIQYVLDQLNRMPAPDYKHLSASQFRSQQHLFPPVKKEPVAEVREFDMDLPGRTLKVRMYRPEGVEPPYPALVYYHGGGWVAGDLETHDPVCRVLAKDGRAVVFSVDYRLAPEHKFPAAVEDAYDALQWIAERAADFHLDPARIAVGGDSAGGNLAAVTSILAKERGGPAIAFQLLIYPFTGYDPAHPPASLLENAEGYLLTGGMMLWFRNQYLNSLEELTHPWFSPVLYPDLSGLPPAYIATAQYDPLRDVGKLYAEALTKAGVKVEIENFEDLIHGFAQFYSLSPGATKALVRIAEKLRDALA

SEQ ID NO: 87 - DNA, 930 bp, synthetic construct
  misc_feature 1..930: note = Description of Artificial Sequence: Syntheticpolynucleotide sequence encoding a codon optimizedcarboxyesterase enzyme
  source 1..930: mol_type = other DNA
atgccattagatcctgtgattcaatatgtcctcgatcaactgaaccgtatgccagcccctgactacaagcacttaagcgctagtcagtttcgttcacagcaacacctgtttccaccagttaagaaagaaccggtcgcagaagttcgcgaattcgacatggatctgccgggccgtaccctgaaagtccgtatgtaccgcccggaaggtgttgaaccaccatatccagcactggtttactaccatggtggcggttgggttgcgggtgacctggaaacgcatgatccggtgtgtcgtgtgttggcgaaagatggacgcgcagtggtgtttagcgttgactaccgtctggcaccagaacacaagtttccagcggcagttgaagacgcgtatgatgcactgcaatggattgcagaacgtgcagccgatttccatcttgatccagcacgcattgcagttggcggcgattcagcaggcggcaacctggcggccgtgactagtattctggcgaaagaacgtggtggtccagcaattgcgtttcaactgctgatctatccctttactggttatgatccagcacatccaccagcaagtcttcttgagaatgcggagggttacctgttaaccggaggcatgatgctgtggtttcgtaatcagtacctgaacagccttgaggaactgactcacccatggtttagtccagtgctgtacccggatcttagcggtttaccaccggcgtacattgcaaccgcacagtacgatcccctgcgcgatgtcggtaaactttacgctgaagccctgaacaaagcgggcgttaaggtggagatcgagaacttcgaggatctgattcatggcttcgcgcagttctattctctgagcccaggcgcaaccaaagcactggtacgtattgccgagaaactgcgcgatgcgttggcg

SEQ ID NO: 88 - protein, 310 aa, synthetic construct
  REGION 1..310: note = Description of Artificial Sequence: Syntheticpolypeptide sequence of a codon optimizedcarboxyesterase enzyme
MPLDPVIQYVLDQLNRMPAPDYKHLSASQFRSQQHLFPPVKKEPVAEVREFDMDLPGRTLKVRMYRPEGVEPPYPALVYYHGGGWVAGDLETHDPVCRVLAKDGRAVVFSVDYRLAPEHKFPAAVEDAYDALQWIAERAADFHLDPARIAVGGDSAGGNLAAVTSILAKERGGPAIAFQLLIYPFTGYDPAHPPASLLENAEGYLLTGGMMLWFRNQYLNSLEELTHPWFSPVLYPDLSGLPPAYIATAQYDPLRDVGKLYAEALNKAGVKVEIENFEDLIHGFAQFYSLSPGATKALVRIAEKLRDALA

SEQ ID NO: 89 - DNA, 930 bp, synthetic construct
  misc_feature 1..930: note = Description of Artificial Sequence: Syntheticpolynucleotide sequence encoding a codon optimizedcarboxyesterase enzyme
  source 1..930: mol_type = other DNA
atgccattagatcctgtgattcaatatgtcctcgatcaactgaaccgtatgccagcccccgactacaagcacttaagcgctcaacaagttcgttcatggcaacacctgtttccaccagttaagaaagaaccggtcgcagaagttcgcgaattcgacatggatctgccgggccgtaccctgaaagtccgtatgtaccgcccggaaggtgttgaaccaccatatcgggcactggtttactaccatggtggcggttgggttgcgggtgacctggaaacgcatgatccggtgtgtcgtgtgttggcgaaatggggacgcgcagtggtgtttagcgttgactaccgtctggcaccagaacacaagtttccagcggcagttgaagacgcgtatgatgcactgcaatggattgcagaacgtgcagccgatttccatcttgatccagcacgcattgcagttggcggcgattcagcaggcggcaacctggcggccgtgactagtattctggcgaaagaacgtggtggtccagcaattgcgtttcaactgctgatctatccctttactggatatgatccagcacatccaccagcaagtatccttgagaatgcggagggttacctgttaaccggaggcatgatgctgtggtttcgtaatcagtacctgaacagccttgaggaactgactcacccatggtttagtccagtgctgtacccggatcttagcggtttaccaccggcgtacattgcaaccgcacagtacgatcccctgcgcgatgtcggcaaactttacgctgaagccctgaacaaagcgggcgttaaagtggagatcgagaacttcgaggatctgattcatggcttcgcgcagttctattctctgagcccaggcgcaaccaaagcactggtacgtattgccgagaaactgcgcgatgcgttggcg

SEQ ID NO: 90 - protein, 310 aa, synthetic construct
  REGION 1..310: note = Description of Artificial Sequence: Syntheticpolypeptide sequence of a codon optimizedcarboxyesterase enzyme
MPLDPVIQYVLDQLNRMPAPDYKHLSAQQVRSWQHLFPPVKKEPVAEVREFDMDLPGRTLKVRMYRPEGVEPPYRALVYYHGGGWVAGDLETHDPVCRVLAKWGRAVVFSVDYRLAPEHKFPAAVEDAYDALQWIAERAADFHLDPARIAVGGDSAGGNLAAVTSILAKERGGPAIAFQLLIYPFTGYDPAHPPASILENAEGYLLTGGMMLWFRNQYLNSLEELTHPWFSPVLYPDLSGLPPAYIATAQYDPLRDVGKLYAEALNKAGVKVEIENFEDLIHGFAQFYSLSPGATKALVRIAEKLRDALA

SEQ ID NO: 91 - DNA, 930 bp, synthetic construct
  misc_feature 1..930: note = Description of Artificial Sequence: Syntheticpolynucleotide sequence encoding a codon optimizedcarboxyesterase enzyme
  source 1..930: mol_type = other DNA
atgccattagatcctgtgattcaatatgtcctcgatcaactgaaccgtatgccagccattgactacaagcacttaagcgctcaacaagttcgttcatggcaacacctgtttccaccagttaagaaagaaccggtccgcgaagttcgcgaattcgacatggatctgccgggccgtaccctgaaagtccgtatgtacacgccggaaggtgttgaaccaccatatccagcactggtttactaccatggtggcggttgggttgcgggtgacctggaaacgcatgatccggtgtgtcgtgtgttggcgaaatggggacgcgcagtggtgtttagcgttgactaccgtctggcaccagaacacaagtttccagcggcagttgaagacgcgtatgatgcactgcaatggattgcagaacgtgcagccgatttccatcttgatccagcacgcattgcagttggcggcgattcagcaggcggcaacctggcggccgtgactagtattctggcgaaagaacgtggtggtccagcaattgcgtttcaactgctgatctatccctttactggatatgatccagcacatccaccagcaagtatccttgagaatgcggagggttacctgttaaccggaggcatgatgctgtggtttcgtaatcagtacctgaacagccttgaggaactgactcacccatggtttagtccagtgctgtacccggatcttagcggtttaccaccggcgtacattgcaaccgcacagtacgatcccctgcgcgatgtcggcaaactttacgctagagccctgaacaaagcgggcgttaaagtggagatcgagaacttcgaggatctgattcatggcttcgcgcagttctattctctgagcccaggcgcaaccaaagcactggtacgtattgccgagaaactgcgcgatgcgttggcg

SEQ ID NO: 92 - protein, 310 aa, synthetic construct
  REGION 1..310: note = Description of Artificial Sequence: Syntheticpolypeptide sequence of a codon optimizedcarboxyesterase enzyme
MPLDPVIQYVLDQLNRMPAIDYKHLSAQQVRSWQHLFPPVKKEPVREVREFDMDLPGRTLKVRMYTPEGVEPPYPALVYYHGGGWVAGDLETHDPVCRVLAKWGRAVVFSVDYRLAPEHKFPAAVEDAYDALQWIAERAADFHLDPARIAVGGDSAGGNLAAVTSILAKERGGPAIAFQLLIYPFTGYDPAHPPASILENAEGYLLTGGMMLWFRNQYLNSLEELTHPWFSPVLYPDLSGLPPAYIATAQYDPLRDVGKLYARALNKAGVKVEIENFEDLIHGFAQFYSLSPGATKALVRIAEKLRDALA

SEQ ID NO: 93 - DNA, 930 bp, synthetic construct
  misc_feature 1..930: note = Description of Artificial Sequence: Syntheticpolynucleotide sequence encoding a codon optimizedcarboxyesterase enzyme
  source 1..930: mol_type = other DNA
atgccattagatcctgtgattcaatatgtcctcgatcaactgaaccgtatgccagcccctgactggaagcacttaagcgctcaacagtttcgttcacagcaacacctgtttccaccagttaagaaagaaccggtcgcagaagttcgcgaattcgacatggatctgccgggccgtaccctgaaagtccgtatgtaccgcccggaaggtgttgaaccaccatatcgggcactggtttactaccatggtggcggttgggttgcgggtgacctggaaacgcatgatccggtgtgtcgtgtgttggcgaaagatggacgcgcagtggtgtttagcgttgactaccgtctggcaccagaacacaagtttccagcggcagttgaagacgcgtatgatgcactgcaatggattgcagaacgtgcagccgatttccatcttgatccagcacgcattgcagttggcggcgattcagcgggcggcaacctggcggccgtgactagtattctggcgaaagaacgtggtggtccagcaattgcgtttcaactgctgatctatccctttactggttatgatccagcacatccaccagcaagtatccttgagaatgcggagggttacctgttaaccggaggcatgatgctgtggtttcgtaatcagtacctgaacagccttgaggaactgactcacccatggtttagtccagtgctgtacccggatcttagcggtttaccaccggcgtacattgcaaccgcacagtacgatcccctgcgcgatgtcggcaaactttacgctgaagccctgaacaaagcgggcgttaaggtggagatcgagaacttcgaggatctgattcatggcttcgcgcagttctattctattagcccaggcgcaaccaaagcactggtacgtattgccgagaaactgcgcgatgcgttggcg

SEQ ID NO: 94 - protein, 310 aa, synthetic construct
  REGION 1..310: note = Description of Artificial Sequence: Syntheticpolypeptide sequence of a codon optimizedcarboxyesterase enzyme
MPLDPVIQYVLDQLNRMPAPDWKHLSAQQFRSQQHLFPPVKKEPVAEVREFDMDLPGRTLKVRMYRPEGVEPPYRALVYYHGGGWVAGDLETHDPVCRVLAKDGRAVVFSVDYRLAPEHKFPAAVEDAYDALQWIAERAADFHLDPARIAVGGDSAGGNLAAVTSILAKERGGPAIAFQLLIYPFTGYDPAHPPASILENAEGYLLTGGMMLWFRNQYLNSLEELTHPWFSPVLYPDLSGLPPAYIATAQYDPLRDVGKLYAEALNKAGVKVEIENFEDLIHGFAQFYSISPGATKALVRIAEKLRDALA

SEQ ID NO: 95 - DNA, 930 bp, synthetic construct
  misc_feature 1..930: note = Description of Artificial Sequence: Syntheticpolynucleotide sequence encoding a codon optimizedcarboxyesterase enzyme
  source 1..930: mol_type = other DNA
atgccattagatcctgtgattcaatatgtcctcgatcaactgaaccgtatgccagcccctgactacaagcacttaagcgctcaacagtttcgttcacagcaacacctgtttccaccagttaagaaagaaccggtcaaagaagttcgcgaattcgacatggatctgccgggccgtaccctgaaagtccgtatgtaccgcccggaaggtgttgaaccaccatatccagcactggtttactaccatggtggcggttgggttgcgggtgacctggaaacgcatgatccggtgtgtcgtgtgttggcgaaagatggacgcgcagtggtgtttagcgttgactaccgtctggcaccagaacacaagtttccagcggcagttgaagacgcgtatgatgcactgcaatggattgcagaacgtgcagccgatttccatcttgatccagcacgcattgcagttggcggcgattcagcaggcggcaacaccgcggccgtgactagtattctggcgaaagaacgtggtggtccagcaattgcgtttcaactgctgatctatccctttactggttatgatccagcacatccaccagcaagtatccttgagaatgcggagggttacctgttaaccggaggcatgatgctgtggtttcgtaatcagtacctgaacagccttgaggaactgactcacccatggtttagtccagtgctgtacccggatcttagcggtttaccaccggcgtacattgcaaccgcacagtacgatcccctgcgcgatgtcggcaaactttacgctgaagccctgaacaaagcgggcgttaaggtggagatcgagaacttcgaggatctgattcatggcttcgcgaacttctattctctgagcccaggcgcaaccaaagcactggtacgtattgccgagaaactgcgcgatgcgttggcg

SEQ ID NO: 96 - protein, 310 aa, synthetic construct
  REGION 1..310: note = Description of Artificial Sequence: Syntheticpolypeptide sequence of a codon optimizedcarboxyesterase enzyme
MPLDPVIQYVLDQLNRMPAPDYKHLSAQQFRSQQHLFPPVKKEPVKEVREFDMDLPGRTLKVRMYRPEGVEPPYPALVYYHGGGWVAGDLETHDPVCRVLAKDGRAVVFSVDYRLAPEHKFPAAVEDAYDALQWIAERAADFHLDPARIAVGGDSAGGNTAAVTSILAKERGGPAIAFQLLIYPFTGYDPAHPPASILENAEGYLLTGGMMLWFRNQYLNSLEELTHPWFSPVLYPDLSGLPPAYIATAQYDPLRDVGKLYAEALNKAGVKVEIENFEDLIHGFANFYSLSPGATKALVRIAEKLRDALA

SEQ ID NO: 97 - DNA, 930 bp, synthetic construct
  misc_feature 1..930: note = Description of Artificial Sequence: Syntheticpolynucleotide sequence encoding a codon optimizedcarboxyesterase enzyme
  source 1..930: mol_type = other DNA
atgccattagatcctgtgattcaatatgtcctcgatcaactgaaccgtatgccagcccctgactacaagcacttaagcgctcaacagtttcgttcacagcaacacctgtttccaccagttaagaaagaaccggtcaaagaagttcgcgaattcgacatggatctgccgggccgtaccctgaaagtccgtatgtaccgcccggaaggtgttgaaccaccatatccagcactggtttactaccatggtggcggttgggttgcgggtgacctggaaacgcatgatccggtgtgtcgtgtgttggcgaaagatggacgcgcagtggtgtttagcgttgactaccgtctggcaccagaacacaagtttccagcggcagttgaagacgcgtatgatgcactgcaatggattgcagaacgtgcagccgatttccatcttgatccagcacgcattgcagttggcggcgattcagcaggcggcaacaccgcggccgtgactagtattctggcgaaagaacgtggtggtccagcaattgcgtttcaactgctgatctatccctttactggttatgatccagcacatccaccagcaagtatccttgagaatgcggagggttacctgttaaccggaggcatgatgctgtggtttcgtaatcagtacctgaacagccttgaggaactgactcacccatggtttagtccagtgctgtacccggatcttagcggtttaccaccggcgtacattgcaaccgcacagtacgatcccctgcgcgatgtcggcaaactttacgctgaagccctgaacaaagcgggcgttaaggtggagatcgagaacttcgaggatctgattcatggcttcgcgagcttctattctctgagcccaggcgcaaccaaagcactggtacgtattgccgagaaactgcgcgatgcgttggcg

SEQ ID NO: 98 - protein, 310 aa, synthetic construct
  REGION 1..310: note = Description of Artificial Sequence: Syntheticpolypeptide sequence of a codon optimizedcarboxyesterase enzyme
MPLDPVIQYVLDQLNRMPAPDYKHLSAQQFRSQQHLFPPVKKEPVKEVREFDMDLPGRTLKVRMYRPEGVEPPYPALVYYHGGGWVAGDLETHDPVCRVLAKDGRAVVFSVDYRLAPEHKFPAAVEDAYDALQWIAERAADFHLDPARIAVGGDSAGGNTAAVTSILAKERGGPAIAFQLLIYPFTGYDPAHPPASILENAEGYLLTGGMMLWFRNQYLNSLEELTHPWFSPVLYPDLSGLPPAYIATAQYDPLRDVGKLYAEALNKAGVKVEIENFEDLIHGFASFYSLSPGATKALVRIAEKLRDALA

SEQ ID NO: 99 - DNA, 930 bp, synthetic construct
  misc_feature 1..930: note = Description of Artificial Sequence: Syntheticpolynucleotide sequence encoding a codon optimizedcarboxyesterase enzyme
  source 1..930: mol_type = other DNA
atgccattagatcctgtgattcaatatgtcctcgatcaactgaaccgtatgccagcccctgactacaagcacttaagcgcttgccagtttcgttcacagcaacacctgtttgaaccagttaagaaagaaccggtcgcagaagttcgcgaattcgacatggatctgccgggccgtaccctgaaagtccgtatgtaccgcccggaaggtgttgaaccaccatatccagcactggtttactaccatggtggcggtggcgttgcgggtgacctggaaacgcatgatccggtgtgtcgtgtgttggcgaaagatggacgcgcagtggtgtttagcgttgactaccgtctggcaccagaacacaagtttccagcggcagttgaagacgcgtatgatgcactgcaatggattgcagaacgtgcagccgatttccatcttgatccagcacgcattgcagttggcggcgattcagcaggcggcaacctggcggccgtgactagtattctggcgaaagaacgtggtggtccagcaattgcgtttcaactgctgatctatccctttactggttatgatccagcacatccaccagcaagtatccttgagaatgcggagggttacctgttaaccggaggcatgatgctgtggtttcgtaatcagtacctgaacagccttgaggaactgactcacccatggtttagtccagtgctgtacccggatcttagcggtttaccaccggcgtacattgcaaccgcacagtacgatcccctgcgcgatgtcggcaaactttacgctgaagccctgaacaaagcgggcgttaaggtggagatcgagaacttcgaggatctgattcatggcttcgcgcagttctattctctgagcccaggcgcaaccaaagcactggtacgtattgccgagaaactgcgcgatgcgttggcg

SEQ ID NO: 100 - protein, 310 aa, synthetic construct
  REGION 1..310: note = Description of Artificial Sequence: Syntheticpolypeptide sequence of a codon optimizedcarboxyesterase enzyme
MPLDPVIQYVLDQLNRMPAPDYKHLSACQFRSQQHLFEPVKKEPVAEVREFDMDLPGRTLKVRMYRPEGVEPPYPALVYYHGGGGVAGDLETHDPVCRVLAKDGRAVVFSVDYRLAPEHKFPAAVEDAYDALQWIAERAADFHLDPARIAVGGDSAGGNLAAVTSILAKERGGPAIAFQLLIYPFTGYDPAHPPASILENAEGYLLTGGMMLWFRNQYLNSLEELTHPWFSPVLYPDLSGLPPAYIATAQYDPLRDVGKLYAEALNKAGVKVEIENFEDLIHGFAQFYSLSPGATKALVRIAEKLRDALA

SEQ ID NO: 101 - DNA, 930 bp, synthetic construct
  misc_feature 1..930: note = Description of Artificial Sequence: Syntheticpolynucleotide sequence encoding a codon optimizedcarboxyesterase enzyme
  source 1..930: mol_type = other DNA
atgccattagatcctgtgattcaatatgtcctcgatcaactgaaccgtatgccagcccctgactacaagcacttaagcgctcaacagtttcgttcacagcaaagcctgtttccaccagttaagaaagaaccggtcgcagaagttcgcgaattcgacatggatctgccgggccgtaccctgaaagtccgtatgtacctgccggaaggtgttgaaccaccatatccagcactggtttactaccatggtggcggttggaccgcgggtgacctggaaacgcatgatccgatgtgtcgtgtgttggcgaaagatggacgcgcagtggtgtttagcgttgactaccgtctggcaccagaacacaagtttccagcggcagttgaagacgcgtatgatgcactgcaatggattgcagaacgtgcagccgatttccatcttgatccagcacgcattgcagttggcggcgattcagcaggcggcaacccggcggccgtgactagtattctggcgaaagaacgtggtggtccagcaattgcgtttcaactgctgatccagccctttactggttttgatccagcacatccaccagcaagtatccttgagaatgcggagggttactttttaaccggaggcatgatggattggtttcgtaatcagtacctgaacagccttgaggaactgactcacccatggtttagtccagtgctgtacccggatcttagcggtttaccaccggcgtacattgcaaccgcacagtacgatcccctgaacgatgtcggcaaactttacgctgaagccctgaacaaagcgggcctgaaggtggagatcgagaacttcgaggatctgattcatggcttcgcgagcttctattctctgagcccaggcgcaaccaaagcactggtacgtattgccgagaaactgcgcgatgcgttggcg

SEQ ID NO: 102 - protein, 310 aa, synthetic construct
  REGION 1..310: note = Description of Artificial Sequence: Syntheticpolypeptide sequence of a codon optimizedcarboxyesterase enzyme
MPLDPVIQYVLDQLNRMPAPDYKHLSAQQFRSQQSLFPPVKKEPVAEVREFDMDLPGRTLKVRMYLPEGVEPPYPALVYYHGGGWTAGDLETHDPMCRVLAKDGRAVVFSVDYRLAPEHKFPAAVEDAYDALQWIAERAADFHLDPARIAVGGDSAGGNPAAVTSILAKERGGPAIAFQLLIQPFTGFDPAHPPASILENAEGYFLTGGMMDWFRNQYLNSLEELTHPWFSPVLYPDLSGLPPAYIATAQYDPLNDVGKLYAEALNKAGLKVEIENFEDLIHGFASFYSLSPGATKALVRIAEKLRDALA

SEQ ID NO: 103 - DNA, 930 bp, synthetic construct
  misc_feature 1..930: note = Description of Artificial Sequence: Syntheticpolynucleotide sequence encoding a codon optimizedcarboxyesterase enzyme
  source 1..930: mol_type = other DNA
atgccattagatcctgtgattcaatatgtcctcgatcaactgaaccgtatgccagcccctgactacaagcacttaagcgctcaacagtttcgttcacagcaaagcctgtttccaccagttaagaaagaaccggtcgcagaagttcgcgaattcgacatggatctgccgggccgtaccctgaaagtccgtatgtacctgccggaaggtgttgaaccaccatatccagcactggtttactaccatggtggcggttggaccgcgggtgacctggaaacgcatgatccgatgtgtcgtgtgttggcgaaagatggacgcgcagtggtgtttagcgttgactaccgtctggcaccagaacacaagtttccagcggcagttgaagacgcgtatgatgcactgcaatggattgcagaacgtgcagccgatttccatcttgatccagcacgcattgcagttggcggcgattcagcaggcggcaacctggcggccgtgactagtattctggcgaaagaacgtggtggtccagcaattgcgtttcaactgctgatctatccctttactggttatgatccagcacatccaccagcaagtatccttgagaatgcggagggttactttttaaccggaggcatgatgctgtggtttcgtaatcagtacctgaacagccttgaggaactgactcacccatggtttagtccagtgctgtacccggatcttagcggtttaccaccggcgtacattgcaacctggcagtacgatcccctgcgcgatgtcggcaaactttacgctgaagccctgaacaaagcgggcgttaaggtggagatcgagaacttcgaggatctgattcatggcttcgcgagcttctattctctgagcccaggcgcaaccaaagcactggtacgtattgccgagaaactgcgcgatgcgttggcg

SEQ ID NO: 104 - protein, 310 aa, synthetic construct
  REGION 1..310: note = Description of Artificial Sequence: Syntheticpolypeptide sequence of a codon optimizedcarboxyesterase enzyme
MPLDPVIQYVLDQLNRMPAPDYKHLSAQQFRSQQSLFPPVKKEPVAEVREFDMDLPGRTLKVRMYLPEGVEPPYPALVYYHGGGWTAGDLETHDPMCRVLAKDGRAVVFSVDYRLAPEHKFPAAVEDAYDALQWIAERAADFHLDPARIAVGGDSAGGNLAAVTSILAKERGGPAIAFQLLIYPFTGYDPAHPPASILENAEGYFLTGGMMLWFRNQYLNSLEELTHPWFSPVLYPDLSGLPPAYIATWQYDPLRDVGKLYAEALNKAGVKVEIENFEDLIHGFASFYSLSPGATKALVRIAEKLRDALA

SEQ ID NO: 105 - DNA, 930 bp, synthetic construct
  misc_feature 1..930: note = Description of Artificial Sequence: Syntheticpolynucleotide sequence encoding a codon optimizedcarboxyesterase enzyme
  source 1..930: mol_type = other DNA
atgccattagatcctgtgattcaatatgtcctcgatcaactgaaccgtatgccagcccctgactacaagcacttaagcgcttgccagtttcgttcacagcaacacctgtttccaccagttaagaaagaaccggtcgcagaagttcgcgaattcgacatgcgtctgccgggccgtaccctgaaagtccgtatgtaccgcccggaaggtgttgaaccaccatatcgtgcactggtttactaccatggtggcggttgggttgcgggtgacctggaaacgcatgatccggtgtgtcgtgtgttggcgaaagatggacgcgcagtggtgtttagcgttgactaccgtctggcaccagaacacaagtttccagcggcagttgaagacgcgtatgatgcactgcaatggattgcagaacgtgcagccgatttccatcttgatccagcacgcattgcagttggcggcgattcagcaggcggcaacctggcggccgtgactagtattctggcgaaagaacgtggtggtccagcaatggcgtttcaactgctgatctatccctttactggttatgatccagcacatccaccagcaagtatccttgagaatgcggagggttactttttaaccggaggcatgatgctgtggtttcgtaatcagtacctgaacagccttgaggaactgactcacccatggtttagtccagtgctgtacccggatcttagcggtttaccaccggcgtacattgcagtggcacagtacgatcccctgcgcgatgtcggcaaactttacgctgaagccctgaacaaagcgggcgttaaggtggagatcgagaacttcgaggatctgattcatggcttcgcgcagttctattctctgagcccaggcgcaaccaaagcactggtacgtattgccgagaaactgcgcgatgcgttggcg

SEQ ID NO: 106 - protein, 310 aa, synthetic construct
  REGION 1..310: note = Description of Artificial Sequence: Syntheticpolypeptide sequence of a codon optimizedcarboxyesterase enzyme
MPLDPVIQYVLDQLNRMPAPDYKHLSACQFRSQQHLFPPVKKEPVAEVREFDMRLPGRTLKVRMYRPEGVEPPYRALVYYHGGGWVAGDLETHDPVCRVLAKDGRAVVFSVDYRLAPEHKFPAAVEDAYDALQWIAERAADFHLDPARIAVGGDSAGGNLAAVTSILAKERGGPAMAFQLLIYPFTGYDPAHPPASILENAEGYFLTGGMMLWFRNQYLNSLEELTHPWFSPVLYPDLSGLPPAYIAVAQYDPLRDVGKLYAEALNKAGVKVEIENFEDLIHGFAQFYSLSPGATKALVRIAEKLRDALA

SEQ ID NO: 107 - DNA, 930 bp, synthetic construct
  misc_feature 1..930: note = Description of Artificial Sequence: Syntheticpolynucleotide sequence encoding a codon optimizedcarboxyesterase enzyme
  source 1..930: mol_type = other DNA
atgccattagatcctgtgcttcaatatgtgctcgatcaactgaaccgtatgccagcccctgactacaagcacttaagcgcttgccagtttcgttcacagcaacacctgtttgaaccagttaagaaagaaccggtcgctgaagttcgcgaattcgacatggacctgccgggccgtaccctgaaagtccgtatgtaccgcccggaaggtgttgaaccaccatatccagcactggtttactaccatggtggcggtggcgttgcgggtgacctggaaacgcatgatccggtgtgtcgtgtgttggcgaaagatggacgcgcagtggtgtttagcgttgactaccgtctggcaccagaacacaagtttccagcggcagttgaagacgcgtatgatgcactgcaatggattgcagaacgtgcagccgatttccatcttgatccagcacgcattgcagttggcggcgattcagcaggcggcaacctcgcggccgtgactagtattctggcgaaagaacgtggtggtccagcaattgcgtttcaactgctgatctatccctttactggttatgatccagcacatccaccagcaagtatcctggagaatgcggagggttacctgttaaccggaggcatgatgctgtggtttcgtaatcagtacctgaacagccttgaggaactgactcacccatggtttagtccagtgctgtacccggatcttagcggtttaccaccggcgtacattgcaaccgcacagtacgatcccctgcgcgatgtcggcaaactttacgctgaagccctgaacaaagcgggcgttaaggtggagatcgagaacttcgaggatctgattcatggcttcgcgcagttctattctctgagcccaggcgcaaccaaagcactggtacgtattgccgagaaactgcgcgatgcgttggcg

SEQ ID NO: 108 - protein, 310 aa, synthetic construct
  REGION 1..310: note = Description of Artificial Sequence: Syntheticpolypeptide sequence of a codon optimizedcarboxyesterase enzyme
MPLDPVLQYVLDQLNRMPAPDYKHLSACQFRSQQHLFEPVKKEPVAEVREFDMDLPGRTLKVRMYRPEGVEPPYPALVYYHGGGGVAGDLETHDPVCRVLAKDGRAVVFSVDYRLAPEHKFPAAVEDAYDALQWIAERAADFHLDPARIAVGGDSAGGNLAAVTSILAKERGGPAIAFQLLIYPFTGYDPAHPPASILENAEGYLLTGGMMLWFRNQYLNSLEELTHPWFSPVLYPDLSGLPPAYIATAQYDPLRDVGKLYAEALNKAGVKVEIENFEDLIHGFAQFYSLSPGATKALVRIAEKLRDALA

SEQ ID NO: 109 - DNA, 930 bp, synthetic construct
  misc_feature 1..930: note = Description of Artificial Sequence: Syntheticpolynucleotide sequence encoding a codon optimizedcarboxyesterase enzyme
  source 1..930: mol_type = other DNA
atgccattagatcctgtgattcaatatgtgctcgatcaactgaaccgtatgccagcccctgactacaagcacttaagcgcttgccagtttcgttcacagcaacacctgtttgaaccagttaagaaagaaccggtcaaagaagttcgcgaattcgacatggacctgccgggccgtaccctgaaagtccgtatgtaccgcccggaaggtgttgaaccaccatatccagcactggtttactaccatggtggcggtggcgttgcgggtgacctggaaacgcatgatccggtgtgtcgtgtgttggcgaaagatggacgcgcagtggtgtttagcgttgactaccgtctggcaccagaacacaagtttccagcggcagttgaagacgcgtatgatgcactgcaatggattgcagaacgtgcagccgatttccatcttgatccagcacgcattgcagttggcggcgattcagcaggcggcaacctcgcggccgtgactagtattctggcgaaagaacgtggtggtccagcaattgcgtttcaactgctgatctatccctttactggttatgatccagcacatccaccagcaagtatccttgagaatgcggagggttacctgttaaccggaggcatgatgctgtggtttcgtaatcagtacctgaacagccttgaggaactgactcacccatggtttagtccagtgctgtacccggatcttagcggtttaccaccggcgtacattgcaaccgcacagtacgatcccctgcgcgatgtcggcaaactttacgctgaagccctgaacaaagcgggcgttaaggtggagatcgagaacttcgaggatctgattcatggcttcgcgcagttctattctctgagcccaggcgcaaccaaagcactggtacgtattgccgagaaactgcgcgatgcgttggcg

SEQ ID NO: 110 - protein, 310 aa, synthetic construct
  REGION 1..310: note = Description of Artificial Sequence: Syntheticpolypeptide sequence of a codon optimizedcarboxyesterase enzyme
MPLDPVIQYVLDQLNRMPAPDYKHLSACQFRSQQHLFEPVKKEPVKEVREFDMDLPGRTLKVRMYRPEGVEPPYPALVYYHGGGGVAGDLETHDPVCRVLAKDGRAVVFSVDYRLAPEHKFPAAVEDAYDALQWIAERAADFHLDPARIAVGGDSAGGNLAAVTSILAKERGGPAIAFQLLIYPFTGYDPAHPPASILENAEGYLLTGGMMLWFRNQYLNSLEELTHPWFSPVLYPDLSGLPPAYIATAQYDPLRDVGKLYAEALNKAGVKVEIENFEDLIHGFAQFYSLSPGATKALVRIAEKLRDALA

SEQ ID NO: 111 - DNA, 930 bp, synthetic construct
  misc_feature 1..930: note = Description of Artificial Sequence: Syntheticpolynucleotide sequence encoding a codon optimizedcarboxyesterase enzyme
  source 1..930: mol_type = other DNA
atgccattagatcctgtgattcaatatgtcctcgatcaactgaaccgtatgccagcccctgactacaagcacttaagcgcttgccagtttcgttcacagcaacacacgttttggccagttaagaaagaaccggtcgcagaagttcgcgaattcgacatgcagctgccgggccgtaccctgaaagtccgtatgtacacgccggaaggtgttgaaccaccatatccagcactggtttactaccatggtggcggtggcgttgcgggtgacctggaaacgcatgatccggtgtgtcgtgtgttggcgaaagatggacgcgcagtggtgtttagcgttgactaccgtctggcaccagaacacaagtttccagcggcagttgaagacgcgtatgatgcactgcaatggattgcagaacgtgcagccgatttccatcttgatccagcacgcattgcagttggcggcgattcagcaggcggcaacctggcggccgtgactagtattctggcgaaagaacgtggtggtccagcaattgcgtttcaactgctgatctatccctttactggttatgatccagcacatccaccagcaagtatccttgagaatgcggagggttacctgttaaccggaggcatgatgctgtggtttcgtaatcagtacctgaacagccttgaggaactgactcacccatggtttagtccagtgctgtacccggatcttagcggtttaccaccggcgtacattgcaaccgcacagtacgatcccctgcgcgatgtcggcaaactttacgctgaagccctgaacaaagcgggcgttaaggtggagatcgagaacttcgaggatctgattcatggcttcgcgcagttctattctctgagcccaggcgcaaccaaagcactggtacgtattgccgagaaactgcgcgatgcgttggcg

SEQ ID NO: 112 - protein, 310 aa, synthetic construct
  REGION 1..310: note = Description of Artificial Sequence: Syntheticpolypeptide sequence of a codon optimizedcarboxyesterase enzyme
MPLDPVIQYVLDQLNRMPAPDYKHLSACQFRSQQHTFWPVKKEPVAEVREFDMQLPGRTLKVRMYTPEGVEPPYPALVYYHGGGGVAGDLETHDPVCRVLAKDGRAVVFSVDYRLAPEHKFPAAVEDAYDALQWIAERAADFHLDPARIAVGGDSAGGNLAAVTSILAKERGGPAIAFQLLIYPFTGYDPAHPPASILENAEGYLLTGGMMLWFRNQYLNSLEELTHPWFSPVLYPDLSGLPPAYIATAQYDPLRDVGKLYAEALNKAGVKVEIENFEDLIHGFAQFYSLSPGATKALVRIAEKLRDALA

SEQ ID NO: 113 - DNA, 930 bp, synthetic construct
  misc_feature 1..930: note = Description of Artificial Sequence: Syntheticpolynucleotide sequence encoding a codon optimizedcarboxyesterase enzyme
  source 1..930: mol_type = other DNA
atgccattagatcctgtgattcaatatgtcctcgatcaactgaaccgtatgccagcccctgactacaagcacttaagcgcttgccagtttcgttcacagcaacacacgttttggccagttaagaaagaaccggtcgcagaagttcgcgaattcgacatggatctgccgggccgtaccctgaaagtccgtatgtaccgcccggaaggtgttgaaccaccatatcgcgcactggtttactaccatggtggcggtggcgttgcgggtgacctggaaacgcatgatccggtgtgtcgtgtgttggcgaaagatggacgcgcagtggtgtttagcgttgactaccgtctggcaccagaacacaagtttccagcggcagttgaagacgcgtatgatgcactgcaatggattgcagaacgtgcagccgatttccatcttgatccagcacgcattgcagttggcggcgattcagcaggcggcaacctggcggccgtgactagtattctggcgaaagaacgtggtggtccagcaattgcgtttcaactgctgatctatccctttactggttatgatccagcacatccaccagcaagtatccttgagaatgcggagggttacctgttaaccggaggcatgatgctgtggtttcgtaatcagtacctgaacagccttgaggaactgactcacccatggtttagtccagtgctgtacccggatcttagcggtttaccaccggcgtacattgcaaccgcacagtacgatcccctgcgcgatgtcggcaaactttacgctgaagccctgaacaaagcgggcgttaaggtggagatcgagaacttcgaggatctgattcatggcttcgcgcagttctattctctgagcccaggcgcaaccaaagcactggtacgtattgccgagaaactgcgcgatgcgttggcg

SEQ ID NO: 114 - protein, 310 aa, synthetic construct
  REGION 1..310: note = Description of Artificial Sequence: Syntheticpolypeptide sequence of a codon optimizedcarboxyesterase enzyme
MPLDPVIQYVLDQLNRMPAPDYKHLSACQFRSQQHTFWPVKKEPVAEVREFDMDLPGRTLKVRMYRPEGVEPPYRALVYYHGGGGVAGDLETHDPVCRVLAKDGRAVVFSVDYRLAPEHKFPAAVEDAYDALQWIAERAADFHLDPARIAVGGDSAGGNLAAVTSILAKERGGPAIAFQLLIYPFTGYDPAHPPASILENAEGYLLTGGMMLWFRNQYLNSLEELTHPWFSPVLYPDLSGLPPAYIATAQYDPLRDVGKLYAEALNKAGVKVEIENFEDLIHGFAQFYSLSPGATKALVRIAEKLRDALA

SEQ ID NO: 115 - DNA, 930 bp, synthetic construct
  misc_feature 1..930: note = Description of Artificial Sequence: Syntheticpolynucleotide sequence encoding a codon optimizedcarboxyesterase enzyme
  source 1..930: mol_type = other DNA
atgccattagatcctgtgattcaatatgtcctcgatcaactgaaccgtatgccagcccctgactggaagcacttaagcgcttgccagtttcgttcacagcaacacatgttttggccagttaagaaagaaccggtcgccgaagttcgcgaattcgacatggatctgccgggccgtaccctgaaagtccgtatgtaccgcccggaaggtgttgaaccaccatatcgcgcactggtttactaccatggtggcggtggcgttgcgggtgacctggaaacgcatgatccggtgtgtcgtgtgttggcgaaagatggacgcgcagtggtgtttagcgttgactaccgtctggcaccagaacacaagtttccagcggcagttgaagacgcgtatgatgcactgcaatggattgcagaacgtgcagccgatttccatcttgatccagcacgcattgcagttggcggcgattcagcaggcggcaacctggcggccgtgactagtattctggcgaaagaacgtggtggtccagcaattgcgtttcaactgctgatctatccctttactggttatgatccagcacatccaccagcaagtatccttgagaatgcggagggttacctgttaaccggaggcatgatgctgtggtttcgtaatcagtacctgaacagccttgaggaactgactcacccatggtttagtccagtgctgtacccggatcttagcggtttaccaccggcgtacattgcaaccgcacagtacgatcccctgcgcgatgtcggcaaactttacgctgaagccctgaacaaagcgggcgttaaggtggagatcgagaacttcgaggatctgattcatggcttcgcgcagttctattctctgagcccaggcgcaaccaaagcactggtacgtattgccgagaaactgcgcgatgcgttggcg

SEQ ID NO: 116 - protein, 310 aa, synthetic construct
  REGION 1..310: note = Description of Artificial Sequence: Syntheticpolypeptide sequence of a codon optimizedcarboxyesterase enzyme
MPLDPVIQYVLDQLNRMPAPDWKHLSACQFRSQQHMFWPVKKEPVAEVREFDMDLPGRTLKVRMYRPEGVEPPYRALVYYHGGGGVAGDLETHDPVCRVLAKDGRAVVFSVDYRLAPEHKFPAAVEDAYDALQWIAERAADFHLDPARIAVGGDSAGGNLAAVTSILAKERGGPAIAFQLLIYPFTGYDPAHPPASILENAEGYLLTGGMMLWFRNQYLNSLEELTHPWFSPVLYPDLSGLPPAYIATAQYDPLRDVGKLYAEALNKAGVKVEIENFEDLIHGFAQFYSLSPGATKALVRIAEKLRDALA

SEQ ID NO: 117 - DNA, 930 bp, synthetic construct
  misc_feature 1..930: note = Description of Artificial Sequence: Syntheticpolynucleotide sequence encoding a codon optimizedcarboxyesterase enzyme
  source 1..930: mol_type = other DNA
atgccattagatcctgtgattcaatatgtcctcgatcaactgaaccgtatgccagcccctgactacaagcacttaagcgcttgccagtttcgttcacagcaacacacgttttggccagttaagaaagaaccggtcgcagaagttcgcgaattcgacatggatctgccgggccgtaccctgaaagtccgtatgtaccgcccggaaggtgttgaaccaccatatatggcactggtttactaccatggtggcggtggcgttgcgggtgacctggaaacgcatgatccggtgtgtcgtgtgttggcgaaagatggacgcgcagtggtgtttagcgttgactaccgtctggcaccagaacacaagtttccagcggcagttgaagacgcgtatgatgcactgcaatggattgcagaacgtgcagccgatttccatcttgatccagcacgcattgcagttggcggcgattcagcaggcggcaacctggcggccgtgactagtattctggcgaaagaacgtggtggtccagcaattgcgtttcaactgctgatctatccctttactggttatgatccagcacatccaccagcaagtatccttgagaatgcggagggttacctgttaaccggaggcatgatgctgtggtttcgtaatcagtacctgaacagccttgaggaactgactcacccatggtttagtccagtgctgtacccggatcttagcggtttaccaccggcgtacattgcaaccgcacagtacgatcccctgcgcgatgtcggcaaactttacgctgaagccctgaacaaagcgggcgttaaggtggagatcgagaacttcgaggatctgattcatggcttcgcgcagttctattctctgagcccaggcgcaaccaaagcactggtacgtattgccgagaaactgcgcgatgcgttggcg

SEQ ID NO: 118 - protein, 310 aa, synthetic construct
  REGION 1..310: note = Description of Artificial Sequence: Syntheticpolypeptide sequence of a codon optimizedcarboxyesterase enzyme
MPLDPVIQYVLDQLNRMPAPDYKHLSACQFRSQQHTFWPVKKEPVAEVREFDMDLPGRTLKVRMYRPEGVEPPYMALVYYHGGGGVAGDLETHDPVCRVLAKDGRAVVFSVDYRLAPEHKFPAAVEDAYDALQWIAERAADFHLDPARIAVGGDSAGGNLAAVTSILAKERGGPAIAFQLLIYPFTGYDPAHPPASILENAEGYLLTGGMMLWFRNQYLNSLEELTHPWFSPVLYPDLSGLPPAYIATAQYDPLRDVGKLYAEALNKAGVKVEIENFEDLIHGFAQFYSLSPGATKALVRIAEKLRDALA

SEQ ID NO: 119 - DNA, 930 bp, synthetic construct
  misc_feature 1..930: note = Description of Artificial Sequence: Syntheticpolynucleotide sequence encoding a codon optimizedcarboxyesterase enzyme
  source 1..930: mol_type = other DNA
atgccattagatcctgtgattcaatatgtcctcgatcaactgaaccgtatgccagcccctgactacaagcacttaagcgcttgccagtttcgttcacagcaacacctgtttgaaccagttaagaaagaaccggtcgcagaagttcgcgaattcgacatggatctgccgggccgtaccctgaaagtccgtatgtaccgcccggaaggtgttgaaccaccatatccagcactggtttactaccatggtggcggtggcgttgcgggtgacctggaaacgcatgatccggtgtgtcgtgtgttggcgaaagatggacgcgcagtggtgtttagcgttgactaccgtctggcaccagaacacaagtttccagcggcagttgaagacgcgtatgatgcactgcaatggattgcagaacgtgcagccgatttccatcttgatccagcacgcattgcagttggcggcgattcagcaggcggcaacctggcggccgtgactagtattctggcgaaagaacgtggtggtccagcaattgcgtttcaactgctgatctatccctttactggttatgatccagcacatccaccagcaagtatccttgagaatgcggagggttacctgttaaccggaggcatgatgctgtggtttcgtaatcagtacctgaacagccttgaggaactgactcacccatggtttagtccagtgctgtacccggatcttagcggtttaccaccggcgtacattgcaaccgcacagtacgatcccctgcgcgatgtcggcaaactttacgctgaagccctgaacaaagcgggcgttaaggtggagatcgagaacttcgaggatctgattcatggcttcgcacagttctattctctgagcccaggcgcaaccaaagcactggtacgtattgccgagaaactgcgcgatgcgttggcg

SEQ ID NO: 120 - protein, 310 aa, synthetic construct; identical to SEQ ID NO: 100
  REGION 1..310: note = Description of Artificial Sequence: Syntheticpolypeptide sequence of a codon optimizedcarboxyesterase enzyme

SEQ ID NO: 121 - DNA, 930 bp, synthetic construct
  misc_feature 1..930: note = Description of Artificial Sequence: Syntheticpolynucleotide sequence encoding a codon optimizedcarboxyesterase enzyme
  source 1..930: mol_type = other DNA
atgccattagatcctgtgattcaatatgtcctcgatcaactgaaccgtatgccagcccctgactacaagcacttaagcgcttgccagtttcgttcacagcaacacacgttttggccagttaagaaagaaccggtcgcagaagttcgcgaattcgacatggatctgccgggccgtaccctgaaagtccgtatgtaccgcccggaaggtgttgaaccaccatatcgcgcactggtttactaccatggtggcggtggcgttgcgggtgacctggaaacgcatgatccggtgtgtcgtgtgttggcgaaagatggacgcgcagtggtgtttagcgttgactaccgtctggcaccagaacacaagtttccagcggcagttgaagacgcgtatgatgcactgcaatggattgcagaacgtgcagccgatttccatcttgatccagcacgcattgcagttggcggcgattcagcaggcggcaacctggcggccgtgactagtattctggcgaaagaacgtggtggtccagcaattgcgtttcaactgctgatctatccctttactggttatgatccagcacatccaccagcaagtatccttgagaatgcggagggttacctgttaaccggaggcatgatgctgtggtttcgtaatcagtacctgaacagccttgaggaactgactcacccatggtttagtccagtgctgtacccggatcttagcggtttaccaccggcgtacattgcaaccgcacagtacgatcccctgcgcgatgtcggcaaactttacgctgaagccctgaacaaagcgggcgttaaggtggagatcgagaacttcgaggatctgattcatggcttcgcgtgtttctattctctgagcccaggcgcaaccaaagcactggtacgtattgccgagaaactgcgcgatgcgttggcg

SEQ ID NO: 122 - protein, 310 aa, synthetic construct
  REGION 1..310: note = Description of Artificial Sequence: Syntheticpolypeptide sequence of a codon optimizedcarboxyesterase enzyme
MPLDPVIQYVLDQLNRMPAPDYKHLSACQFRSQQHTFWPVKKEPVAEVREFDMDLPGRTLKVRMYRPEGVEPPYRALVYYHGGGGVAGDLETHDPVCRVLAKDGRAVVFSVDYRLAPEHKFPAAVEDAYDALQWIAERAADFHLDPARIAVGGDSAGGNLAAVTSILAKERGGPAIAFQLLIYPFTGYDPAHPPASILENAEGYLLTGGMMLWFRNQYLNSLEELTHPWFSPVLYPDLSGLPPAYIATAQYDPLRDVGKLYAEALNKAGVKVEIENFEDLIHGFACFYSLSPGATKALVRIAEKLRDALA

SEQ ID NO: 123 - DNA, 930 bp, synthetic construct
  misc_feature 1..930: note = Description of Artificial Sequence: Syntheticpolynucleotide sequence encoding a codon optimizedcarboxyesterase enzyme
  source 1..930: mol_type = other DNA
atgttgttagatcctgtgattcaatatgtcctcgatcaactgaaccgtatgccagcccctgactacaagcacttaagcgcttgccagtttcgttcacagcaacacacgttttggccagttaagaaagaaccggtcgcagaagttcgcgaattcgacatggatctgccgggccgtaccctgaaagtccgtatgtaccgcccggaaggtgttgaaccaccatatcgcgcactggtttactaccatggtggcggtggcgttgcgggtgacctggaaacgcatgatccggtgtgtcgtgtgttggcgaaagatggacgcgcagtggtgtttagcgttgactaccgtctggcaccagaacacaagtttccagcggcagttgaagacgcgtatgatgcactgcaatggattgcagaacgtgcagccgatttccatcttgatccagcacgcattgcagttggcggcgattcagcaggcggcaacctggcggccgtgactagtattctggcgaaagaacgtggtggtccagcaattgcgtttcaactgctgatctatccctttactggttatgatccagcacatccaccagcaagtatccttgagaatgcggagggttacctgttaaccggaggcatgatgctgtggtttcgtaatcagtacctgaacagccttgaggaactgactcacccatggtttagtccagtgctgtacccggatcttagcggtttaccaccggcgtacattgcaaccgcacagtacgatcccctgcgcgatgtcggcaaactttacgctgaagccctgaacaaagcgggcgttaaggtggagatcgagaacttcgaggatctgattcatggcttcgcgcagttctattctctgagcccaggcgcaaccaaagcactggtacgtattgccgagaaactgcgcgatgcgttggcg

SEQ ID NO: 124 - protein, 310 aa, synthetic construct
  REGION 1..310: note = Description of Artificial Sequence: Syntheticpolypeptide sequence of a codon optimizedcarboxyesterase enzyme
MLLDPVIQYVLDQLNRMPAPDYKHLSACQFRSQQHTFWPVKKEPVAEVREFDMDLPGRTLKVRMYRPEGVEPPYRALVYYHGGGGVAGDLETHDPVCRVLAKDGRAVVFSVDYRLAPEHKFPAAVEDAYDALQWIAERAADFHLDPARIAVGGDSAGGNLAAVTSILAKERGGPAIAFQLLIYPFTGYDPAHPPASILENAEGYLLTGGMMLWFRNQYLNSLEELTHPWFSPVLYPDLSGLPPAYIATAQYDPLRDVGKLYAEALNKAGVKVEIENFEDLIHGFAQFYSLSPGATKALVRIAEKLRDALA

SEQ ID NO: 125 - DNA, 930 bp, synthetic construct
  misc_feature 1..930: note = Description of Artificial Sequence: Syntheticpolynucleotide sequence encoding a codon optimizedcarboxyesterase enzyme
  source 1..930: mol_type = other DNA
atgccattagatcctgtgattcaatatgtcctcgatcaactgaaccgtatgccagcccctgactacaagcacttaagcgcttgccagtttcgttcacagcaacacacgttttggccagttaagaaagaaccggtcgcagaagttcgcgaattcgacatggatctgccgggccgtaccctgaaagtccgtatgtaccgcccggaaggtgttgaaccaccatatcgcgcactggtttactaccatggtggcggtggcgttgcgggtgacctggaaacgcatgatccggtgtgtcgtgtgttggcgaaagatggacgcgcagtggtgtttagcgttgactaccgtctggcaccagaacacaagtttccagcggcagttgaagacgcgtatgatgcactgcaatggattgcagaacgtgcagccgatttccatcttgatccagcacgcattgcagttggcggcgattcagcaggcggcaacctggcggccgtgactagtattctggcgaaagaacgtggtggtccagcaattgcgtttcaactgcaaatctatccctttactggttatgatccagcacatccaccagcaagtatccttgagaatgcggagggttacctgttaaccggaggcatgatgctgtggtttcgtaatcagtacctgaacagccttgaggaactgactcacccatggtttagtccagtgctgtacccggatcttagcggtttaccaccggcgtacattgcaaccgcacagtacgatcccctgcgcgatgtcggcaaactttacgctgaagccctgaacaaagcgggcgttaaggtggagatcgagaacttcgaggatctgattcatggcttcgcgcagttctattctctgagcccaggcgcaaccaaagcactggtacgtattgccgagaaactgcgcgatgcgttggcg

SEQ ID NO: 126 - protein, 310 aa, synthetic construct
  REGION 1..310: note = Description of Artificial Sequence: Syntheticpolypeptide sequence of a codon optimizedcarboxyesterase enzyme
MPLDPVIQYVLDQLNRMPAPDYKHLSACQFRSQQHTFWPVKKEPVAEVREFDMDLPGRTLKVRMYRPEGVEPPYRALVYYHGGGGVAGDLETHDPVCRVLAKDGRAVVFSVDYRLAPEHKFPAAVEDAYDALQWIAERAADFHLDPARIAVGGDSAGGNLAAVTSILAKERGGPAIAFQLQIYPFTGYDPAHPPASILENAEGYLLTGGMMLWFRNQYLNSLEELTHPWFSPVLYPDLSGLPPAYIATAQYDPLRDVGKLYAEALNKAGVKVEIENFEDLIHGFAQFYSLSPGATKALVRIAEKLRDALA